European Patent Specification EP 3 720 458 B1, published July 15, 2026. Title: METHODS AND COMPOSITIONS TO PREVENT MICROBIAL INFECTION. Applicant: BioPlx, Inc. Starzl, Timothy W. Turner, Todd D. Starzl, Ravi S.V. Application New Filing. The sequence listing filed with the application follows.

SEQUENCE LISTING (339 sequences)

SEQ ID NO: 1 - DNA, 1536 bp, Staphylococcus aureus
atgactttacaaatacatacagggggtattaatttgaaaaagaaaaacatttattcaattcgtaaactaggtgtaggtattgcatctgtaactttaggtacattacttatatctggtggcgtaacacctgctgcaaatgctgcgcaacacgatgaagctcaacaaaatgctttttatcaagtgttaaatatgcctaacttaaacgctgatcaacgtaatggttttatccaaagccttaaagatgatccaagccaaagtgctaacgttttaggtgaagctcaaaaacttaatgactctcaagctccaaaagctgatgcgcaacaaaataacttcaacaaagatcaacaaagcgccttctatgaaatcttgaacatgcctaacttaaacgaagcgcaacgtaacggcttcattcaaagtcttaaagacgacccaagccaaagcactaatgttttaggtgaagctaaaaaattaaacgaatctcaagcaccgaaagctgataacaatttcaacaaagaacaacaaaatgctttctatgaaatcttgaatatgcctaacttaaacgaagaacaacgcaatggtttcatccaaagcttaaaagatgacccaagccaaagtgctaacctattgtcagaagctaaaaagttaaatgaatctcaagcaccgaaagcggataacaaattcaacaaagaacaacaaaatgctttctatgaaatcttacatttacctaacttaaacgaagaacaacgcaatggtttcatccaaagcttaaaagatgacccaagccaaagcgctaaccttttagcagaagctaaaaagctaaatgatgcacaagcaccaaaagctgacaacaaattcaacaaagaacaacaaaatgctttctatgaaattttacatttacctaacttaactgaagaacaacgtaacggcttcatccaaagccttaaagacgatccttcagtgagcaaagaaattttagcagaagctaaaaagctaaacgatgctcaagcaccaaaagaggaagacaacaaaaaacctggtaaagaagacggcaacaagcctggtaaagaagacaacaaaaaacctggtaaagaagacggcaacaagcctggtaaagaagacaacaacaaacctggcaaagaagacggcaacaagcctggtaaagaagacaacaacaagcctggtaaagaagacggcaacaagcctggtaaagaagacggcaacaaacctggtaaagaagacggcaacggagtacatgtcgttaaacctggtgatacagtaaatgacattgcaaaagcaaacggcactactgctgacaaaattgctgcagataacaaattagctgataaaaacatgatcaaacctggtcaagaacttgttgttgataagaagcaaccagcaaaccatgcagatgctaacaaagctcaagcattaccagaaactggtgaagaaaatccattcatcggtacaactgtatttggtggattatcattagccttaggtgcagcgttattagctggacgtcgtcgcgaactataa

SEQ ID NO: 2 - DNA, 993 bp, Staphylococcus aureus
atgaataaagtaattaaaatgcttgttgttacgcttgctttcctacttgttttagcaggatgtagtgggaattcaaataaacaatcatctgataacaaagataaggaaacaacttcaattaaacatgcaatgggtacaactgaaattaaagggaaaccaaagcgtgttgttacgctatatcaaggtgccactgacgtcgctgtatctttaggtgttaaacctgtaggtgctgtagaatcatggacacaaaaaccgaaattcgaatacataaaaaatgatttaaaagatactaagattgtaggtcaagaacctgcacctaacttagaggaaatctctaaattaaaaccggacttaattgtcgcgtcaaaagttagaaatgaaaaagtttacgatcaattatctaaaatcgcaccaacagtttctactgatacagttttcaaattcaaagatacaactaagttaatggggaaagctttagggaaagaaaaagaagctgaagatttacttaaaaagtacgatgataaagtagctgcattccaaaaagatgcaaaagcaaagtataaagatgcatggccattgaaagcttcagttgttaacttccgtgctgatcatacaagaatttatgctggtggatatgctggtgaaatcttaaatgatttaggattcaaacgtaataaagacttacaaaaacaagttgataatggtaaagatattatccaacttacatctaaagaaagcattccattaatgaacgctgatcatatttttgtagtaaaatcagatccaaatgcgaaagatgctgcattagttaaaaagactgaaagcgaatggacttcaagtaaagagtggaaaaatttagacgcagttaaaaacaaccaagtatctgatgatttagatgaaatcacttggaacttagctggcggatataaatcttcattaaaacttattgacgatttatatgaaaagttaaatattgaaaaacaatcaaaataa

SEQ ID NO: 3 - DNA, 1014 bp, Staphylococcus aureus
atgataatgattatcattaatttaaagggagaaaaatttgtaatgaagtatttattaaagggaaatattttgcttctattactaatattgttgacaattatttcgttgttcataggtgtgagtgaactatcaattaaagatttactacatttaactgaatcacagcggaatattttattctcaagccgaataccaaggacgatgagtattttaattgctggaagttcgttggctttagcaggcttgataatgcaacaaatgatgcaaaataagtttgttagtccgactacagctggaacgatggaatgggctaaactaggtattttaattgctttattgttctttccaaccggtcatattttattaaaactagtatttgctgttatttgcagtatttgcggtacgtttttatttgttaaaatcattgattttataaaagtgaaagatgtcatttttgtaccgcttttaggaattatgatgggtgggattgttgcaagtttcacaaccttcatctcattgcgcacgaatgctgttcaaagcattggtaactggcttaacgggaactttgccattatcacaagtggacgctatgaaattttatatttaagtattcctcttttagcattgacatatctttttgctaatcatttcacgattgtaggaatgggtaaagactttactaataatttaggtttgagttacgaaaaattaattaacatcgcattgtttattactgcaactattacagcattggtagtggtgactgttggaacattaccgttcttaggactagtaataccaaatattatttcaatttatcgaggtgatcatttgaaaaatgctatccctcatacgatgatgttaggtgccatctttgtattattttctgatatagttggcagaattgttgtttatccatatgaaataaatattggtttaacaataggtgtatttggaacaatcattttccttatcttgcttatgaaaggtaggaaaaattatgcgcaacaataa

SEQ ID NO: 4 - DNA, 909 bp, Staphylococcus aureus
acagcaactttagcagttggtttaatagcccctttagccaatccatttatagaaatttctaaagcagaaaataagatagaagatatcggtcaaggtgcagaaatcatcaaaagaacacaagacattactagcaaacgattagctataactcaaaacattcaatttgattttgtaaaagataaaaaatataacaaagatgccctagttgttaagatgcaaggcttcatcagctctagaacaacatattcagacttaaaaaaatatccatatattaaaagaatgatatggccatttcaatataatatcagtttgaaaacgaaagactctaatgttgatttaatcaattatcttcctaaaaataaaattgattcagcagatgttagtcagaaattaggctataatatcggcggaaacttccaatcagcgccatcaatcggaggcagtggctcattcaactactctaaaacaattagttataatcaaaaaaactatgttactgaagtagaaagtcagaactctaaaggtgttaaatggggagtgaaagcaaattcatttgttacaccgaatggtcaagtatctgcatatgatcaatacttatttgcacaagacccaactggtccagcagcaagagactatttcgtcccagataatcaattacctcctttaattcaaagtggctttaatccatcatttattacaacattgtcacacgaaagaggtaaaggtgataaaagcgagtttgaaatcacttacggcagaaacatggatgctacatatgcttacgtgacaagacatcgtttagccgttgatagaaaacatgatgcttttaaaaaccgaaacgttacagttaaatatgaagtgaactggaaaacacatgaagtaaaaattaaaagcatcacacctaagtaa

SEQ ID NO: 5 - DNA, 1053 bp, Staphylococcus aureus
atgacaaaacattatttaaacagtaagtatcaatcagaacaacgttcatcagctatgaaaaagattacaatgggtacagcatctatcattttaggttcccttgtatacataggcgcagacagccaacaagtcaatgcggcaacagaagctacgaacgcaactaataatcaaagcacacaagtttctcaagcaacatcacaaccaattaatttccaagtgcaaaaagatggctcttcagagaagtcacacatggatgactatatgcaacaccctggtaaagtaattaaacaaaataataaatattatttccaaaccgtgttaaacaatgcatcattctggaaagaatacaaattttacaatgcaaacaatcaagaattagcaacaactgttgttaacgataataaaaaagcggatactagaacaatcaatgttgcagttgaacctggatataagagcttaactactaaagtacatattgtcgtgccacaaattaattacaatcatagatatactacgcatttggaatttgaaaaagcaattcctacattagctgacgcagcaaaaccaaacaatgttaaaccggttcaaccaaaaccagctcaacctaaaacacctactgagcaaactaaaccagttcaacctaaagttgaaaaagttaaacctactgtaactacaacaagcaaagttgaagacaatcactctactaaagttgtaagtactgacacaacaaaagatcaaactaaaacacaaactgctcatacagttaaaacagcacaaactgctcaagaacaaaataaagttcaaacacctgttaaagatgttgcaacagcgaaatctgaaagcaacaatcaagctgtaagtgataataaatcacaacaaactaacaaagttacaaaacataacgaaacgcctaaacaagcatctaaagctaaagaattaccaaaaactggtttaacttcagttgataactttattagcacagttgccttcgcaacacttgcccttttaggttcattatctttattacttttcaaaagaaaagaatctaaataa

SEQ ID NO: 6 - DNA, 1527 bp, Staphylococcus aureus
atgagtagtcatattcaaatttttgatacgacactaagagacggtgaacaaacaccaggagtgaattttacttttgatgaacgcttgcgtattgcattgcaattagaaaaatggggtgtagatgttattgaagctggatttcctgcttcaagtacaggtagctttaaatctgttcaagcaattgcacaaacattaacaacaacggctgtatgtggtttagctagatgtaaaaaatctgacatcgatgctgtatatgaagcaacaaaagatgcagcgaagccggtcgtgcatgtttttatagcaacatcacctattcatcttgaacataaacttaaaatgtctcaagaagacgttttagcatctattaaagaacatgtcacatacgcgaaacaattatttgacgttgttcaattttcacctgaagatgcaacgcgtactgaattaccattcttagtgaaatgtgtacaaactgccgttgacgctggagctacagttattaatattcctgatacagtcggctacagttaccatgatgaatatgcacatattttcaaaaccttaacagaatctgtaacatcttcaaatgaaattatttatagtgctcattgccatgacgatttaggaatggctgtttcaaatagtttagctgcaattgaaggcggtgcgagacgaattgaaggcactgtaaatggtattggtgaacgagcaggtaatgcagcacttgaagaagtcgcgcttgcactatacgttcgaaatgatcattatggtgctcaaactgcccttaatctcgaagaaactaaaaaaacatcggatttaatttcaagatatgcaggtattcgagtgcctagaaataaagcaattgttggccaaaatgcatttagtcatgaatcaggtattcaccaagatggcgtattaaaacatcgtgaaacatatgaaattatgacacctcaacttgttggtgtaagcacgactgaacttccattaggaaaattatctggtaaacacgccttctcagagaagttaaaagcattaggttataacattgataaagaagcgcaaatagatttatttaaacaattcaagaccattgcggacaaaaagaaatctgtttcagatagagatattcatgcgattattcaaggttctgagcatgagcatcaagcactttataaattggaaacactacaactacaatatgtctctagcggccttcaaagtgctgttgttgttgttaaagataaagagggtcatatttaccaggattcaagtattggtactggttcaatcgtagcaatttacaatgcagttgatcgtattttccagaaagaaacagaattaattgattatcgtattaattctgtcactgaaggtactgatgcccaagcagaagtacatgtaaatttattgattgaaggtaagactgtcaatggctttggtattgatcatgatattttacaagcctcttgtaaagcatacgtagaagcacatgctaaatttgcagctgaaaatgttgagaaggtaggtaat

SEQ ID NO: 7 - DNA, 2700 bp, Staphylococcus aureus
atgaaaaaaagaattgattatttgtcgaataagcagaataagtattcgattagacgttttacagtaggtaccacatcagtaatagtaggggcaactatactatttgggataggcaatcatcaagcacaagcttcagaacaatcgaacgatacaacgcaatcttcgaaaaataatgcaagtgcagattccgaaaaaaacaatatgatagaaacacctcaattaaatacaacggctaatgatacatctgatattagtgcaaacacaaacagtgcgaatgtagatagcacaacaaaaccaatgtctacacaaacgagcaataccactacaacagagccagcttcaacaaatgaaacacctcaaccgacggcaattaaaaatcaagcaactgctgcaaaaatgcaagatcaaactgttcctcaagaagcaaattctcaagtagataataaaacaacgaatgatgctaatagcatagcaacaaacagtgagcttaaaaattctcaaacattagatttaccacaatcatcaccacaaacgatttccaatgcgcaaggaactagtaaaccaagtgttagaacgagagctgtacgtagtttagctgttgctgaaccggtagtaaatgctgctgatgctaaaggtacaaatgtaaatgataaagttacggcaagtaatttcaagttagaaaagactacatttgaccctaatcaaagtggtaacacatttatggcggcaaattttacagtgacagataaagtgaaatcaggggattattttacagcgaagttaccagatagtttaactggtaatggagacgtggattattctaattcaaataatacgatgccaattgcagacattaaaagtacgaatggcgatgttgtagctaaagcaacatatgatatcttgactaagacgtatacatttgtctttacagattatgtaaataataaagaaaatattaacggacaattttcattacctttatttacagaccgagcaaaggcacctaaatcaggaacatatgatgcgaatattaatattgcggatgaaatgtttaataataaaattacttataactatagttcgccaattgcaggaattgataaaccaaatggcgcgaacatttcttctcaaattattggtgtagatacagcttcaggtcaaaacacatacaagcaaacagtatttgttaaccctaagcaacgagttttaggtaatacgtgggtgtatattaaaggctaccaagataaaatcgaagaaagtagcggtaaagtaagtgctacagatacaaaactgagaatttttgaagtgaatgatacatctaaattatcagatagctactatgcagatccaaatgactctaaccttaaagaagtaacagaccaatttaaaaatagaatctattatgagcatccaaatgtagctagtattaaatttggtgatattactaaaacatatgtagtattagtagaagggcattacgacaatacaggtaagaacttaaaaactcaggttattcaagaaaatgttgatcctgtaacaaatagagactacagtattttcggttggaataatgagaatgttgtacgttatggtggtggaagtgctgatggtgattcagcagtaaatccgaaagacccaactccagggccgccggttgacccagaaccaagtccagacccagaaccagaaccaacgccagatccagaaccaagtccagacccagaaccggaaccaagcccagacccggatccggattcggattcagacagtgactcaggctcagacagcgactcaggttcagatagcgactcagaatcagatagcgattcggattcagacagtgattcagattcagacagcgactcagaatcagatagcgattcagaatcagatagcgactcagattcagatagcgattcagattcagatagcgattcagaatcagatagcgattcggattcagacagtgattcagattcagacagcgactcagaatcagatagcgactcagaatcagatagtgagtcagattcagacagtgactcggactcagacagtgattcagactcagatagcgattcagactcagatagcgattcagactcagacagcgattcagattcagacagcgactcagaatcagacagcgactcagactcagatagcgactcagactcagacagcgactcagattcagatagcgattcagactcagacagcgactcagactcagacagcgactcagactcagatagcgattcagactcagacagcgactcagattcagatagcgattcggactcagacagcgattcagattcagacagcgactcagactcggatagcgattcagattcagacagcgactcagactcggatagcgactcggattcagatagtgactccgattcaagagttacaccaccaaataatgaacagaaagcaccatcaaatcctaaaggtgaagtaaaccattctaataaggtatcaaaacaacacaaaactgatgctttaccagaaacaggagataagagcgaaaacacaaatgcaactttatttggtgcaatgatggcattattaggatcattactattgtttagaaaacgcaagcaagatcataaagaaaaagcgtaaatacttttttaggccgaatacatttgtattcggtttttttgttgaaaatgattttaaagtgaattg

SEQ ID NO: 8 - DNA, 2673 bp, Staphylococcus aureus
atggctgaattacctcaatcaagaataaatgaacgaaatattaccagtgaaatgcgtgaatcatttttagattatgcgatgagtgttatcgttgctcgtgcattgccagatgttcgtgacggtttaaaaccagtacatcgtcgtatactatatggattaaatgaacaaggtatgacaccggataaatcatataaaaaatcagcacgtatcgttggtgacgtaatgggtaaatatcaccctcatggtgactcatctatttatgaagcaatggtacgtatggctcaagatttcagttatcgttatccgcttgttgatggccaaggtaactttggttcaatggatggagatggcgcagcagcaatgcgttatactgaagcgcgtatgactaaaatcacacttgaactgttacgtgatattaataaagatacaatagattttatcgataactatgatggtaatgaaagagagccgtcagtcttacctgctcgattccctaacttgttagccaatggagcatcaggtatagcggtaggtatggcaacgaatattccaccacataacttaacagaattaatcaatggtgtacttagcttaagtaagaaccctgatatttcaattgctgagttaatggaggatattgaaggtcctgatttcccaactgctggacttattttaggtaagagtggtattagacgtgcatatgaaacaggtcgtggttcaattcaaatgcgttctcgtgcagttattgaagaacgtggaggcggacgtcaacgtattgttgtcactgaaattcctttccaagtgaataaggctcgtatgattgaaaaaattgcagagctcgttcgtgacaagaaaattgacggtatcactgatttacgtgatgaaacaagtttacgtactggtgtgcgtgtcgttattgatgtgcgtaaggatgcaaatgctagtgtcattttaaataacttatacaaacaaacacctcttcaaacatcatttggtgtgaatatgattgcacttgtaaatggtagaccgaagcttattaatttaaaagaagcgttggtacattatttagagcatcaaaagacagttgttagaagacgtacgcaatacaacttacgtaaagctaaagatcgtgcccacattttagaaggattacgtatcgcacttgaccatatcgatgaaattatttcaacgattcgtgagtcagatacagataaagttgcaatggaaagcttgcaacaacgcttcaaactttctgaaaaacaagctcaagctattttagacatgcgtttaagacgtctaacaggtttagagagagacaaaattgaagctgaatataatgagttattaaattatattagtgaattagaaacaatcttagctgatgaagaagtattactacaattagttagagatgaattaacagaaattcgagatcgtttcggtgatgatcgtcgtactgaaatccaattaggtggatttgaagatttagaagatgaagatctcattccagaagaacaaattgtaattacactaagccataataactacattaaacgtttgccggtatctacatatcgtgctcaaaaccgtggtggtcgtggtgttcaaggtatgaatacattggaagaagattttgtcagtcaattggtaactttaagtacacatgaccatgtattgttctttactaacaaaggtcgtgtatacaaacttaaaggttatgaagtgcctgagttatcaagacagtctaaaggtattcctgtagtgaatgctattgaacttgaaaatgatgaagtcattagtacaatgattgctgttaaagaccttgaaagtgaagacaacttcttagtgtttgcaactaaacgtggtgtcgttaaacgttcagcattaagtaacttctcaagaataaatagaaatggtaagattgcgatttcgttcagagaagatgatgagttaattgcagttcgcttaacaagtggtcaagaagatatcttgattggtacatcacatgcatcattaattcgattccctgaatcaacattacgtcctttaggccgtacagcaacgggtgtgaaaggtattacacttcgtgaaggtgacgaagttgtagggcttgatgtagctcatgcaaacagtgttgatgaagtattagtagttactgaaaatggttatggtaaacgtacgccagttaatgactatcgtttatcaaatcgtggtggtaaaggtattaaaacagctacgattactgagcgtaatggtaatgttgtatgtatcactacagtaactggtgaagaagatttaatgattgttactaatgcaggtgtcattattcgactagatgttgcagatatttctcaaaatggtcgtgcagcacaaggtgttcgcttaattcgcttaggtgatgatcaatttgtttcaacggttgctaaagtaaaagaagatgcagaagatgaaacgaatgaagatgagcaatctacttcaactgtatctgaagatggtactgaacaacaacgtgaagcggttgtaaatgatgaaacaccaggaaatgcaattcatactgaagtgattgattcagaagaaaatgatgaagatggacgtattgaagtaagacaagatttcatggatcgtgttgaagaagatatacaacaatcatcagatgaagatgaagaataataa

SEQ ID NO: 9 - DNA, 29 bp, Artificial Sequence
  Primer; TKO1; leuA PCR Amplification with Sph1; upstream pr
gatgcgcatgcgaaacagattatctattc

SEQ ID NO: 10 - DNA, 29 bp, Artificial Sequence
  Primer; TKO2; LeuA PCR Amplification with Sph1 (upstream pr-alternate)
gatgcgcatgccagattatctattcaaag

SEQ ID NO: 11 - DNA, 32 bp, Artificial Sequence
  Primer; TKO3; LeuA PCR Amplification with Pst1 (downstream pr)
catgatctgcagagtaaattcccccgtaaatt

SEQ ID NO: 12 - DNA, 32 bp, Artificial Sequence
  Primer; TKO4; LeuA PCR Amplification with Pst1 (downstream pr-alternate)
cacgtgatctgcagagtaaattcccccgtaaa

SEQ ID NO: 13 - DNA, 32 bp, Artificial Sequence
  Primer; TKO5; upstream primer to amplify ClfB promoter with EcoRI
gactacgaattcaggtgatgaaaaatttagaa

SEQ ID NO: 14 - DNA, 32 bp, Artificial Sequence
  Primer; TKO6; backup upstream primer to amplify ClfB promoter with EcoRI
gactacgaattctgatgaaaaatttagaactt

SEQ ID NO: 15 - DNA, 32 bp, Artificial Sequence
  Primer; TKO7; downstream primer to amplify ClfB promoter with BamHI
cttagctggatccaaatattactccatttcaa

SEQ ID NO: 16 - DNA, 36 bp, Artificial Sequence
  Primer; TKO8; backup downstream primer to amplify ClfB promoter with BamHI
cttagctggatccaaatattactccatttcaatttc

SEQ ID NO: 17 - DNA, 31 bp, Artificial Sequence
  Primer; TKO9; upstream primer to amplify the hlgA RR; contains Sph1
gatgcgcatgctcacaaactattgcgaaatc

SEQ ID NO: 18 - DNA, 32 bp, Artificial Sequence
  Primer; TKO10; backup upstream primer to amplify the hlgA RR
gatgcgcatgcaaactattgcgaaatccattc

SEQ ID NO: 19 - DNA, 32 bp, Artificial Sequence
  Primer; TKO11; downstream primer to amplify hlgA RR; contains pstI
catgatctgcagatatataataatccatttgt

SEQ ID NO: 20 - DNA, 37 bp, Artificial Sequence
  Primer; TKO12; backup downstream primer to amplify hlgA RR
catgatctgcagatatataataatccatttgtaagcg

SEQ ID NO: 21 - DNA, 20 bp, Artificial Sequence
  Primer; TKO13; First sense primer for sequencing constructs containing pCAD promoter
gtgttacgatagcaaatgca

SEQ ID NO: 22 - DNA, 20 bp, Artificial Sequence
  Primer; TKO14; second sense sequencing primer anneals roughly in the middle of the SprA1 gene
ttattggctaagtagacgca

SEQ ID NO: 23 - DNA, 20 bp, Artificial Sequence
  Primer; TKO15; primer to anneal just upstream of the serum responsive RRs for leuA and hlgA. Anneals in the PCN51 vector about 75 nt upstream of the Sph1 site
cacatgttctttcctgcgtt

SEQ ID NO: 24 - DNA, 20 bp, Artificial Sequence
  Primer; TKO16; backup primer to anneal just upstream of the serum responsive RRs for leuA and hlgA
acgcggcctttttacggttc

SEQ ID NO: 25 - DNA, 20 bp, Artificial Sequence
  Primer; TKO17; primer to anneal near the downstream one third of the leuA promoter/RR
gaatgggacttgtaaacgtc

SEQ ID NO: 26 - DNA, 18 bp, Artificial Sequence
  Primer; TKO18; backup primer to anneal near the downstream one third of the leuA promoter/RR
gaatgggacttgtaaacg

SEQ ID NO: 27 - DNA, 20 bp, Artificial Sequence
  Primer; TKO19; primer to anneal near the downstream one third of the hlgA promoter/RR
ataaacgcctgcgaccaata

SEQ ID NO: 28 - DNA, 20 bp, Artificial Sequence
  Primer; TKO20; backup primer to anneal near the downstream one third of the hlgA promoter/RR
gcgaccaataaatcttttaa

SEQ ID NO: 29 - DNA, 40 bp, Artificial Sequence
  Primer; TKO21; pTK1 vector with leuA pro homology R
ttgaatagataatctgtttcgcatgcagcggccgccagct

SEQ ID NO: 30 - DNA, 40 bp, Artificial Sequence
  Primer; TKO22; pTK1 vector with leuA pro homology F
aatttacgggggaatttactctgcagggtaccgcagagag

SEQ ID NO: 31 - DNA, 49 bp, Artificial Sequence
  Primer; TKO23; leuA insert with pTK1 homology F
agctggcggccgctgcatgcgaaacagattatctattcaaagttaattg

SEQ ID NO: 32 - DNA, 46 bp, Artificial Sequence
  Primer; TKO24; leuA insert with pTK1 homology R
ctctctgcggtaccctgcagagtaaattcccccgtaaattttaatg

SEQ ID NO: 33 - DNA, 46 bp, Artificial Sequence
  Primer; TKO25; pTK9 vector with leuA pro homology F
cattaaaatttacgggggaatttactctgcagatgagcagggatga

SEQ ID NO: 34 - DNA, 49 bp, Artificial Sequence
  Primer; TKO26; pTK9 vector with leuA pro homology R
caattaactttgaatagataatctgtttcgcatgcagcggccgccagct

SEQ ID NO: 35 - DNA, 46 bp, Artificial Sequence
  Primer; TKO27; pTK12 vector with leuA pro homology F
cattaaaatttacgggggaatttactctgcagatggtagagatagc

SEQ ID NO: 36 - DNA, 46 bp, Artificial Sequence
  Primer; TKO28; leuA insert with pTK12 homology R
gctatctctaccatctgcagagtaaattcccccgtaaattttaatg

SEQ ID NO: 37 - DNA, 49 bp, Artificial Sequence
  Primer; TKO29; pTKvector R with kanR homology
gcaatccatcttgttcaatcattataaccctctttaatttggttatatg

SEQ ID NO: 38 - DNA, 44 bp, Artificial Sequence
  Primer; TKO30; pTKvector F with kanR homology
ccttcttgacgagttcttctgagttaagggatgcataaactgca

SEQ ID NO: 39 - DNA, 49 bp, Artificial Sequence
  Primer; TKO31; pCASSA kanR F with pTK homology
catataaccaaattaaagagggttataatgattgaacaagatggattgc

SEQ ID NO: 40 - DNA, 44 bp, Artificial Sequence
  Primer; TKO32; pCASSA kanR R with pTK homology
tgcagtttatgcatcccttaactcagaagaactcgtcaagaagg

SEQ ID NO: 41 - DNA, 22 bp, Artificial Sequence
  Primer; TKO33; leuA colony screen PCR F
gaatgggacttgtaaacgtccc

SEQ ID NO: 42 - DNA, 22 bp, Artificial Sequence
  Primer; TKO34; leuA colony screen PCR R
gggacgtttacaagtcccattc

SEQ ID NO: 43 - DNA, 24 bp, Artificial Sequence
  Primer; BPC - T1.1  - FOR; gRNA insertion for pCasSA
gaaaggagtaatatcgatggagta

SEQ ID NO: 44 - DNA, 24 bp, Artificial Sequence
  Primer; BPC - T1.1  - REV; gRNA insertion for pCasSA
caaatactccatcgatattactcc

SEQ ID NO: 45 - DNA, 24 bp, Artificial Sequence
  Primer; gRNA insertion for pCasSA
gaaaggagaggatgatgattataa

SEQ ID NO: 46 - DNA, 24 bp, Artificial Sequence
  Primer; BPC - T1.2  - REV; gRNA insertion for pCasSA
caaattataatcatcatcctctcc

SEQ ID NO: 47 - DNA, 24 bp, Artificial Sequence
  Primer; BPC - T1.3 - FOR; gRNA insertion for pCasSA
gaaagggagaggatgatgattata

SEQ ID NO: 48 - DNA, 24 bp, Artificial Sequence
  Primer; BPC - T1.3 - REV; gRNA insertion for pCasSA
caaatataatcatcatcctctccc

SEQ ID NO: 49 - DNA, 24 bp, Artificial Sequence
  Primer; BPC - T1.4 - FOR; gRNA insertion for pCasSA
gaaagggtctaatgttattgctta

SEQ ID NO: 50 - DNA, 24 bp, Artificial Sequence
  Primer; BPC - T1.4 - REV; gRNA insertion for pCasSA
caaataagcaataacattagaccc

SEQ ID NO: 51 - DNA, 23 bp, Artificial Sequence
  Primer; BPC - T1.5 - FOR; gRNA insertion for pCasSA
gaaaggagaggatgatgattata

SEQ ID NO: 52 - DNA, 23 bp, Artificial Sequence
  Primer; BPC - T1.5 - REV; gRNA insertion for pCasSA
caaatataatcatcatcctctcc

SEQ ID NO: 53 - DNA, 24 bp, Artificial Sequence
  Primer; BPC - T1.6 - FOR; gRNA insertion for pCasSA
gaaaggtagtatgagtaatatcga

SEQ ID NO: 54 - DNA, 24 bp, Artificial Sequence
  Primer; BPC - T1.6 - REV; gRNA insertion for pCasSA
caaatcgatattactcatactacc

SEQ ID NO: 55 - DNA, 24 bp, Artificial Sequence
  Primer; BPC - T1.7 - FOR; gRNA insertion for pCasSA
gaaaggaattatataaatataaag

SEQ ID NO: 56 - DNA, 24 bp, Artificial Sequence
  Primer; BPC - T1.7 - REV; gRNA insertion for pCasSA
caaactttatatttatataattcc

SEQ ID NO: 57 - DNA, 24 bp, Artificial Sequence
  Primer; BPC - T1.8 - FOR; gRNA insertion for pCasSA
gaaaggctacctccatattttcta

SEQ ID NO: 58 - DNA, 24 bp, Artificial Sequence
  Primer; BPC - T1.8 - REV; gRNA insertion for pCasSA
caaatagaaaatatggaggtagcc

SEQ ID NO: 59 - DNA, 24 bp, Artificial Sequence
  Primer; BPC - T1.9 - FOR; gRNA insertion for pCasSA
gaaaggatagaactgtattagact

SEQ ID NO: 60 - DNA, 24 bp, Artificial Sequence
  Primer; BPC - T1.9 - REV; gRNA insertion for pCasSA
caaaagtctaatacagttctatcc

SEQ ID NO: 61 - DNA, 24 bp, Artificial Sequence
  Primer BPC - T1.10 - FOR; gRNA insertion for pCasSA
gaaaggtgtctaatgttattgctt

SEQ ID NO: 62 - DNA, 24 bp, Artificial Sequence
  Primer; BPC - T1.10 - REV; gRNA insertion for pCasSA
caaaaagcaataacattagacacc

SEQ ID NO: 63 - DNA, 20 bp, Artificial Sequence
  Primer; BPC - gRNA - FOR; sequencing primer for gRNA insertion into the pCasSA vector
tgttctttcctgcgttgtcg

SEQ ID NO: 64 - DNA, 24 bp, Artificial Sequence
  Primer; BPC - gRNA - REV; sequencing primer for gRNA insertion into the pCasSA vector
tcgcattgacgttaatacctacat

SEQ ID NO: 65 - DNA, 24 bp, Artificial Sequence
  Primer; BPC - T1.1.2 - REV; reverse primer for gRNA
aaactactccatcgatattactcc

SEQ ID NO: 66 - DNA, 24 bp, Artificial Sequence
  Primer; BPC - T1.2.2 - REV; reverse primer for gRNA
aaacttataatcatcatcctctcc

SEQ ID NO: 67 - DNA, 24 bp, Artificial Sequence
  Primer BPC - T1.3.2 - REV; reverse primer for gRNA
aaactataatcatcatcctctccc

SEQ ID NO: 68 - DNA, 24 bp, Artificial Sequence
  Primer; BPC - T1.4.2 - REV; reverse primer for gRNA
aaactaagcaataacattagaccc

SEQ ID NO: 69 - DNA, 23 bp, Artificial Sequence
  Primer; BPC - T1.5.2 - REV; reverse primer for gRNA
aaactataatcatcatcctctcc

SEQ ID NO: 70 - DNA, 24 bp, Artificial Sequence
  Primer; BPC - T1.6.2 - REV; reverse primer for gRNA
aaactcgatattactcatactacc

SEQ ID NO: 71 - DNA, 24 bp, Artificial Sequence
  Primer; BPC - T1.7.2 - REV; reverse primer for gRNA
aaacctttatatttatataattcc

SEQ ID NO: 72 - DNA, 24 bp, Artificial Sequence
  Primer; BPC - T1.8.2 - REV; reverse primer for gRNA
aaactagaaaatatggaggtagcc

SEQ ID NO: 73 - DNA, 24 bp, Artificial Sequence
  Primer; BPC - T1.9.2 - REV; reverse primer for gRNA
aaacagtctaatacagttctatcc

SEQ ID NO: 74 - DNA, 24 bp, Artificial Sequence
  Primer; BPC - T1.10.2 - REV; reverse primer for gRNA
aaacaagcaataacattagacacc

SEQ ID NO: 75 - DNA, 20 bp, Artificial Sequence
  Primer; BPC - pCN51-1 - FOR; Primer to check insertion into pCN51
tttgctggccttttgctcac

SEQ ID NO: 76 - DNA, 24 bp, Artificial Sequence
  Primer; BPC - pCN51-1 - REV; Primer to check insertion into pCN51
tgctttttcgattgatgaacacct

SEQ ID NO: 77 - DNA, 20 bp, Artificial Sequence
  Primer; BPC - pCN51-2 - FOR; Primer to check insertion into pCN51
cggcctttttacggttcctg

SEQ ID NO: 78 - DNA, 24 bp, Artificial Sequence
  Primer; BPC - pCN51-2 - REV; Primer to check insertion into pCN51
acgttgctttttcgattgatgaac

SEQ ID NO: 79 - DNA, 33 bp, Artificial Sequence
  Primer; BPC - mChr-1 - FOR; mCherry mRNA with Pst1
cacgtgatctgcagtcacatggtgagcaagggc

SEQ ID NO: 80 - DNA, 33 bp, Artificial Sequence
  Primer; BPC - mChr-1 - REV; mCherry mRNA with EcoR1
gactacgaattcaaaactgatttcgttgacccg

SEQ ID NO: 81 - DNA, 34 bp, Artificial Sequence
  Primer; BPC - mChr-2 - REV; mCherry mRNA with BamH1
cttagctggatccaaaactgatttcgttgacccg

SEQ ID NO: 82 - DNA, 37 bp, Artificial Sequence
  Primer; BPC - pCN51-hdr - REV; 34BPC-REV with Xma1, use with TKO15 to add homologous arms
cttagctcccgggtgctttttcgattgatgaacacct

SEQ ID NO: 83 - DNA, 20 bp, Artificial Sequence
  Primer; BPC - 2a - FOR; 502a Target 1 genomic incorp check
cgccaaacgtttcgtcagtt

SEQ ID NO: 84 - DNA, 20 bp, Artificial Sequence
  Primer; BPC - 2a - REV; 502a Target 1 genomic incorp check
ttcaagcgtgacaaagcagc

SEQ ID NO: 85 - DNA, 20 bp, Artificial Sequence
  Primer; BPC - 2a - FOR; 502a Target 1 genomic incorp check
tgcgcaatggccaaaaagat

SEQ ID NO: 86 - DNA, 20 bp, Artificial Sequence
  Primer; BPC - 2a - REV; 502a Target 1 genomic incorp check
cgtgctaacatccgcttcaa

SEQ ID NO: 87 - DNA, 21 bp, Artificial Sequence
  Primer; BPC - mChr-1 - REV; mCherry
aaaactgatttcgttgacccg

SEQ ID NO: 88 - DNA, 33 bp, Artificial Sequence
  Primer; BPC - mChr-1 - FOR; mCherry with Pst1
cacgtgatctgcagtcacatggtttctaaaggt

SEQ ID NO: 89 - DNA, 22 bp, Artificial Sequence
  Primer; BPC - pJ204-1 - FOR; Checking for insertion btwn HAs in pJ204
acgttgctttttcgattgatga

SEQ ID NO: 90 - DNA, 19 bp, Artificial Sequence
  Primer; Checking for insertion btwn HAs in pJ204; Checking for insertion btwn HAs in pJ204
tccccatgcgagagtaggg

SEQ ID NO: 91 - DNA, 23 bp, Artificial Sequence
  Primer; BPC - pJ204-2 - FOR; Checking for insertion btwn HAs in pJ204
gaatatttaagggcgcctgtcac

SEQ ID NO: 92 - DNA, 18 bp, Artificial Sequence
  Primer; BPC - pJ204-2 - REV; Checking for insertion btwn HAs in pJ204
tatggggtgtcgcccttt

SEQ ID NO: 93 - DNA, 19 bp, Artificial Sequence
  Primer; BPC - mChr-1 - FOR; mCherry codon opt seq in pJ204: 300995
tcacatggtttctaaaggt

SEQ ID NO: 94 - DNA, 20 bp, Artificial Sequence
  Primer; BP - repF-1 - F; Checking for repF removal
catgcctgcagaacggattg

SEQ ID NO: 95 - DNA, 20 bp, Artificial Sequence
  Primer; BP - repF-1 - R; Checking for repF removal
gcgcgggaatatgatgctaa

SEQ ID NO: 96 - DNA, 20 bp, Artificial Sequence
  Primer; BP - repF-2 - F; Checking for repF removal
aggtgactgatggctggttg

SEQ ID NO: 97 - DNA, 20 bp, Artificial Sequence
  Primer; BP - repF-2 - R; Checking for repF removal
tatgtcttttgcgcagtcgg

SEQ ID NO: 98 - DNA, 24 bp, Artificial Sequence
  Primer; BP - srtA - F; srtA CRISPR targeting from Dong et al.
gaaacaaacaaatatgctgccact

SEQ ID NO: 99 - DNA, 24 bp, Artificial Sequence
  Primer; BP - srtA - R; srtA CRISPR targeting
aaacagtggcagcatatttgtttg

SEQ ID NO: 100 - DNA, 24 bp, Artificial Sequence
  Primer; BP - hla - F; hla CRISPR targeting from Dong et al.
gaaagcttccaatatctgtagtac

SEQ ID NO: 101 - DNA, 24 bp, Artificial Sequence
  Primer; BP - hla - R; BP - hla - R
aaacgtactacagatattggaagc

SEQ ID NO: 102 - DNA, 24 bp, Artificial Sequence
  Primer; BP - coa - F; coa CRISPR targeting from Dong et al.
gaaagccatttttaaatctgtacg

SEQ ID NO: 103 - DNA, 24 bp, Artificial Sequence
  Primer; BP  - coa - R; coa CRISPR targeting
aaaccgtacagatttaaaaatggc

SEQ ID NO: 104 - protein, 30 aa, Staphylococcus aureus
MLIFVHIIAPVISGCAIAFFSYWLSRRNTK

SEQ ID NO: 105 - protein, 31 aa, Artificial Sequence
  pepA1- related antimicrobial peptide; WO 2013/050590
MMLIFVHIIAPVISGCAIAFFSYWLSRRNTK

SEQ ID NO: 106 - protein, 15 aa, Artificial Sequence
  pepA1- related antimicrobial peptide; WO 2013/050590
AIAFFSYWLSRRNTK

SEQ ID NO: 107 - protein, 14 aa, Artificial Sequence
  pepA1- related antimicrobial peptide; WO 2013/050590
IAFFSYWLSRRNTK

SEQ ID NO: 108 - protein, 13 aa, Artificial Sequence
  pepA1- related antimicrobial peptide; WO 2013/050590
AFFSYWLSRRNTK

SEQ ID NO: 109 - protein, 12 aa, Artificial Sequence
  pepA1- related antimicrobial peptide; WO 2013/050590
FFSYWLSRRNTK

SEQ ID NO: 110 - protein, 11 aa, Artificial Sequence
  pepA1- related antimicrobial peptide; WO 2013/050590
FSYWLSRRNTK

SEQ ID NO: 111 - protein, 10 aa, Artificial Sequence
  pepA1- related antimicrobial peptide; WO 2013/050590
SYWLSRRNTK

SEQ ID NO: 112 - protein, 9 aa, Artificial Sequence
  pepA1- related antimicrobial peptide; WO 2013/050590
YWLSRRNTK

SEQ ID NO: 113 - protein, 33 aa, Staphylococcus aureus
MQGFKEKHQELKKALCQIGLMRSISEVKQLNIA

SEQ ID NO: 114 - DNA, 402 bp, Staphylococcus aureus
gcatgcgaaacagattatctattcaaagttaattgtaagaaaatttaaaatatttgttgacatactaaagcagatatagtaaattaaatttatcaaatttttagacaattctaactattaaagtgatatataccattcacggaaggagtataataaaatgcttaatcaatatactgaacatcaaccgacaacttcaaatattattattttattatactctttaggactcgaacgttagtaaatatttactaaacgctttaagtcctatttctgtttgaatgggacttgtaaacgtcccaataatattgggacgtttttttatgttttatctttcaattacttatttttattactataaaacatgattaatcattaaaatttacgggggaatttactctgcag

SEQ ID NO: 115 - DNA, 297 bp, Staphylococcus aureus
gcatgcaaactattgcgaaatccattcctcttccactacaagcaccataattaaacaacaattcaatagaataagacttgcaaaacatagttatgtcgctatataaacgcctgcgaccaataaatcttttaaacataacataatgcaaaaacatcatttaacaatgctaaaaatgtctcttcaatacatgttgatagtaattaacttttaacgaacagttaattcgaaaacgcttacaaatggattattatatatatgaacttaaaattaaatagaaagaaagtgatttctctgcag

SEQ ID NO: 116 - DNA, 598 bp, Artificial Sequence
  Promoter; Cadmium promoter sequence between restriction sites SphI and PstI
gcatgcgcacttattcaagtgtattttttaataaattattttacttattgaaatgtattattttctaatgtcataccctggtcaaaaccgttcgtttttgagactagaattttatgccctacttacttcttttattttcattcaaatatttgcttgcatgatgagtcgaaaatggttataatacactcaaataaatatttgaatgaagatgggatgataatatgaaaaagaaagatacttgtgaaattttttgttatgacgaagaaaaggttaatcgaatacaaggggatttacaaacagttgatatttctggtgttagccaaattttaaaggctattgccgatgaaaatagagcaaaaattacttacgctctgtgtcaggatgaagagttgtgtgtttgtgatatagcaaatatcttaggtgttacgatagcaaatgcatctcatcatttacgtacgctttataagcaaggggtggtcaactttagaaaagaaggaaaactagctttatattctttaggtgatgaacatatcaggcagataatgatgatcgccctagcacataagaaagaagtgaaggtcaatgtctgaacctgcag

SEQ ID NO: 117 - DNA, 231 bp, Artificial Sequence
  Promoter; clfB promoter forward sequence with EcoRI and BamHI sites
gaattcaggtgatgaaaaatttagaacttctaagtttttgaaaagtaaaaaatttgtaatagtgtaaaaatagtatattgatttttgctagttaacagaaaattttaagttatataaataggaagaaaacaaattttacgtaatttttttcgaaaagcaattgatataattcttatttcattatacaatttagactaatctagaaattgaaatggagtaatatttggatcc

SEQ ID NO: 118 - DNA, 231 bp, Artificial Sequence
  Promoter; clfB promoter as it is cloned in pCN51 vector with EcoRI and BamHI reversed
ggatccaaatattactccatttcaatttctagattagtctaaattgtataatgaaataagaattatatcaattgcttttcgaaaaaaattacgtaaaatttgttttcttcctatttatataacttaaaattttctgttaactagcaaaaatcaatatactatttttacactattacaaattttttacttttcaaaaacttagaagttctaaatttttcatcacctgaattc

SEQ ID NO: 119 - DNA, 303 bp, Staphylococcus aureus
ttagaaagatttacttttatatatgaagagactggattaaatacttttattgacgtaaaaattcacttttgaaccgttcaatatcttgccgatttttatataacagctacaaataaaatataacagtttgattttacagcctcggtaaatcgtcttgacaaacaaaaattttgtgctatcacaacatttgcaacgtcttaacaagtcatctataaacatttctaaatatttaacattacttatgcgtcatttattgctaaaattattgtattaaaatatacatagaattgatgggatatcatg

SEQ ID NO: 120 - DNA, 303 bp, Staphylococcus aureus
acgaaaaattaattaacatcgcattgtttattactgcaactattacagcattggtagtggtgactgttggaacattaccgttcttaggactagtaataccaaatattatttcaatttatcgaggtgatcatttgaaaaatgctatccctcatacgatgatgttaggtgccatctttgtattattttctgatatagttggcagaattgttgtttatccatatgaaataaatattggtttaacaataggtgtatttggaacaatcattttccttatcttgcttatgaaaggtaggaaaaattatg

SEQ ID NO: 121 - DNA, 303 bp, Staphylococcus aureus
ctatctgcggcatttgcagaattactgaatgtcgcgatgatgataattaacgctaaaatcgttgtattaaaaacttttaaaatatttttcaaaacataatcctcctttttatgattgcttttaagtctttagtaaaatcataaataataatgattatcattgtcaatatttattttataatcaatttattattgttatacggaaatagatgtgctagtataattgataaccattatcaattgcaatggttaatcatctcatataacaacacataatttgtatccttaggaggaaaacaacatg

SEQ ID NO: 122 - DNA, 233 bp, Artificial Sequence
  ORF for sprA1 for plasmid construction
ctgcagggtaccgcagagaggaggtgtataaggtgatgcttattttcgttcacatcatagcaccagtcatcagtggctgtgccattgcgtttttttcttattggctaagtagacgcaatacaaaataggtgacatatagccgcaccaataaaaatcccctcactaccgcaaatagtgaggggattggtgtataagtaaatacttattttcgttgtggatccttgactgaattc

SEQ ID NO: 123 - DNA, 233 bp, Artificial Sequence
  DNA sequence for the regulatory RNA sprA1sprA1AS (sprA1sprA1 antisense) under the ClfB promoter which is cloned in reverse behind the sprA1 gene, including the antisense regulatory RNA
gaattcagtcaaggatccacaacgaaaataagtatttacttatacaccaatcccctcactatttgcggtagtgaggggatttttattggtgcggctatatgtcacctattttgtattgcgtctacttagccaataagaaaaaaacgcaatggcacagccactgatgactggtgctatgatgtgaacgaaaataagcatcaccttatacacctcctctctgcggtaccctgcag

SEQ ID NO: 124 - DNA, 756 bp, Artificial Sequence
  SmaI DNA sequence between restriction sites PstI and EcoRI
ctgcagatgagcagggatgaccaactctttacactttggggaaagcttaacgatcgtcagaaggataattttctaaaatggatgaaagcttttgatgtagagaaaacttaccaaaaaacaagtggggatattttcaatgatgattttttcgatatatttggtgatagattaattactcatcatttcagtagcacgcaagctttaacaaaaactttattcgaacatgcttttaatgactccttaaatgaatctggagttatatcctctcttgcggaaagtagaacaaaccctgggcatgacataacaatcgatagcataaaggttgctttaaaaacagaagcagctaaaaatattagcaaatcatatattcatgtaagtaagtggatggagttaggcaagggggagtggattctagaattattattagaacggtttttagagcatctagagaattatgaacgtattttcacactcagatattttaaaatatccgagtataaatttagctaccagcttgtagaaatacccaagagtcttttgttggaagcaaaaaatgcgaaattagaaataatgtcgggaagcaaacaaagccctaagcccggctatggatatgtgttagatgaaaatgaaaataagaagttttctctatactttgatggtggtgccgagagaaaacttcaaataaaacatttaaatttagaacattgcattgttcatggagtttgggattttattctaccgccgccttaagaattc

SEQ ID NO: 125 - DNA, 142 bp, Artificial Sequence
  rsaE DNA sequence between restriction sites PstI and EcoRI
ctgcagatggtagagatagcatgttatattatgaacatgaaattaatcacataacaaacatacccctttgtttgaagtgaaaaatttctcccatcccctttgtttagcgtcgtgtattcagacacgacgtttttttgaattc

SEQ ID NO: 126 - DNA, 104 bp, Artificial Sequence
  Variant can be used for RsaE sRNA which may express the sRNA
gaaattaatcacataacaaacatacccctttgtttgaagtgaaaaatttctcccatcccctttgtttagcgtcgtgtattcagacacgacgtttttttgaattc

SEQ ID NO: 127 - DNA, 156 bp, Escherichia coli
atgaagcagcaaaaggcgatgttaatcgccctgatcgtcatctgtttaaccgtcatagtgacggcactggtaacgaggaaagacctctgcgaggtacgaatccgaaccggccagacggaggtcgctgtcttcacagcttacgaacctgaggagtaa

SEQ ID NO: 128 - DNA, 657 bp, Klebsiella pneumoniae
atggatgtctttgataaagtttatagtgatgataataatagttatgaccaaaaaactgtaagtcagcgtattgaagccctatttcttaataaccttggcaaagttgtaactcgtcagcaaatcattagggcggcaactgatccaaaaacagggaaacaaccagaaaattggcatcagagactttcagaactacgaactgataaaggatatactattttatcctggcgggatatgaaggttttagctccgcaagagtatataatgccacacgcaacaagacgcccaaaggcagcaaagcgtgtattaccgacaaaagaaacctgggaacaggttttggatagagctaattactcttgcgagtggcaggaagatggtcaacactgtgggttagttgaaggtgatattgatcctatagggggaggcacggtcaaactaacaccagaccatatgacacctcattcaatagatcccgcaactgatgtaaatgatcctaaaatgtggcaagcattgtgtggacgtcatcaagttatgaaaaaaaattattgggattcaaataatgggaaaataaatgtcattggtatattgcagtcagtaaatgagaaacaaaagaatgatgctttagagtttcttttgaattattatggattgaaaagataa

SEQ ID NO: 129 - DNA, 219 bp, Artificial Sequence
  Promoter; clfB promoter F downregulated in serum
aggtgatgaaaaatttagaacttctaagtttttgaaaagtaaaaaatttgtaatagtgtaaaaatagtatattgatttttgctagttaacagaaaattttaagttatataaataggaagaaaacaaattttacgtaatttttttcgaaaagcaattgatataattcttatttcattatacaatttagactaatctagaaattgaaatggagtaatattt

SEQ ID NO: 130 - DNA, 219 bp, Artificial Sequence
  Promoter; clfB promoter R downregulated in serum
tccactactttttaaatcttgaagattcaaaaacttttcattttttaaacattatcacatttttatcatataactaaaaacgatcaattgtcttttaaaattcaatatatttatccttcttttgtttaaaatgcattaaaaaaagcttttcgttaactatattaagaataaagtaatatgttaaatctgattagatctttaactttacctcattataaa

SEQ ID NO: 131 - DNA, 5743 bp, Artificial Sequence
  Plasmid; pIMAY Integrative Plasmid accession number JQ62198
gcatgcgttttagcgtttatttcgtttagttatcggcataatcgttaaaacaggcgttatcgtagcgtaaaagcccttgagcgtagcgtggctttgcagcgaagatgttgtctgttagattatgaaagccgatgactgaatgaaataataagcgcagcgcccttctatttcggttggaggaggctcaagggagtatgagggaatgaaattccctcatgggtttgattttaaaaattgcttgcaattttgccgagcggtagcgctggaaaatttttgaaaaaaatttggaatttggaaaaaaatggggggaaaggaagcgaattttgcttccgtactacgaccccccattaagtgccgagtgccaatttttgtgccaaaaacgctctatcccaactggctcaagggtttaaggggtttttcaatcgccaacgaatcgccaacgttttcgccaacgttttttataaatctatatttaagtagctttattgttgtttttatgattacaaagtgatacactaactttataaaattatttgattggagttttttaaatggtgatttcagaatcgaaaaaaagagttatgatttctctgacaaaagagcaagataaaaaattaacagatatggcgaaacaaaaaggtttttcaaaatctgcggttgcggcgttagctatagaagaatatgcaagaaaggaatcagaacaaaaaaaataagcgaaagctcgcgtttttagaaggatacgagttttcgctacttgtttttgataaggtaattatatcatggctattaaaaatactaaagctagaaattttggatttttattatatcctgactcaattcctaatgattggaaagaaaaattagagagtttgggcgtatctatggctgtcagtcctttacacgatatggacgaaaaaaaagataaagatacatggaataatagtaatattatacaaaatggaaagcactataaaaaaccacactatcacgttatatatattgcacgaaatcctgtaacaatagaaagcgttaggaacaagattaagcgaaaattggggaatagttcagttgctcatgttgagatacttgattatatcaaaggttcatatgaatatttgactcatgaatcaaaggacgctattgctaagaataaacatatatacgacaaaaaagatattttgaacattaatgattttgatattgaccgctatataacacttgatgaaagccaaaaaagagaattgaagaatttacttttagatatagtggatgactataatttggtaaatacaaaagatttaatggcttttattcgccttaggggagcggagtttggaattttaaatacgaatgatgtaaaagatattgtttcaacaaactctagcgcctttagattatggtttgagggcaattatcagtgtggatatagagcaagttatgcaaaggttcttgatgctgaaacgggggaaataaaatgacaaacaaagaaaaagagttatttgctgaaaatgaggaattaaaaaaagaaattaaggacttaaaagagcgtattgaaagatacagagaaatggaagttgaattaagtacaacaatagatttattgagaggagggattattgaataaataaaagccccctgacgaaagtcgaagggggtttttattttggtttgatgttgcgattaatagcaatacattctataatagaaggtatggaggatgttatataatgagacagaattatgatgatcatatgtcaactaacggggcaggttagtgacattagaaaaccgactgtaaaaagtacagtcggcattatctcatattataaaagccagtcattaggcctatctgacaattcctgaatagagttcataaacaatcctgcatgataaccatcacaaacagaatgatgtacctgtaaagatagcggtaaatatattgaattacctttattaatgaattttcctgctgtaataatgggtagaaggtaattactattattattgatatttaagttaaacccagtaaatgaagtccatggaataatagaaagagaaaaagcattttcaggtataggtgttttgggaaacaatttccccgaaccattatatttctctacatcagaaaggtataaatcataaaactctttgaagtcattctttacaggagtccaaataccagagaatgttttagatacaccatcaaaaattgtataaagtggctctaacttatcccaataacctaactctccgtcgctattgtaaccagttctaaaagctgtatttgagtttatcacccttgtcactaagaaaataaatgcagggtaaaatttatatccttcttgttttatgtttcggtataaaacactaatatcaatttctgtggttatactaaaagtcgtttgttggttcaaataatgattaaatatctcttttctcttccaattgtctaaatcaattttattaaagttcatgggtttcactctccttctacattttttaacctaataatgccaaataccgtttgccacccctctctttgataattataatattggcgaaattcgcttctaaagatgaaacgcaatattatatgcttgctttatcggccgtatgtgattataccagccccctcactacatgtcaagaataaactgccaaagcataatgggataattaaccctcactaaagggaacaaaagctgggtaccgggccccccctcgaggtcgacggtatcgataagcttgatatcgaattcctgcagcccgggggatccactagttctagagcggccgccaccgcggtggagctccaattcgccctatagtgagtcgtattacgacgtcccagggcttcccggtatcaacagggacaccaggatttatttattctgcgaagtgatcttccgtcacaggtatttattcggcgcaaagtgcgtcgggtgatgctgccaacttactgatttagtgtatgatggtgtttttgaggtgctccagtggcttctgtttctatcagctgtccctcctgttcagctactgacggggtggtgcgtaacggcaaaagcaccgccggacatcagcgctagcggagtgtatactggcttactatgttggcactgatgagggtgtcagtgaagtgcttcatgtggcaggagaaaaaaggctgcaccggtgcgtcagcagaatatgtgatacaggatatattccgcttcctcgctcactgactcgctacgctcggtcgttcgactgcggcgagcggaaatggcttacgaacggggcggagatttcctggaagatgccaggaagatacttaacagggaagtgagagggccgcggcaaagccgtttttccataggctccgcccccctgacaagcatcacgaaatctgacgctcaaatcagtggtggcgaaacccgacaggactataaagataccaggcgtttccccctggcggctccctcgtgcgctctcctgttcctgcctttcggtttaccggtgtcattccgctgttatggccgcgtttgtctcattccacgcctgacactcagttccgggtaggcagttcgctccaagctggactgtatgcacgaaccccccgttcagtccgaccgctgcgccttatccggtaactatcgtcttgagtccaacccggaaagacatgcaaaagcaccactggcagcagccactggtaattgatttagaggagttagtcttgaagtcatgcgccggttaaggctaaactgaaaggacaagttttggtgactgcgctcctccaagccagttacctcggttcaaagagttggtagctcagagaaccttcgaaaaaccgccctgcaaggcggttttttcgttttcagagcaagagattacgcgcagaccaaaacgatctcaagaagatcatcttattaatcagataaaatatttctagatttcagtgcaatttatctcttcaaatgtagcacctgaagtcagccccatacgatataagttgtaattctccgccgcttgccctcatctgttacgccggcggtagccggccagcctcgcagagcaggattcccgttgagcaccgccaggtgcgaataagggacagtgaagaaggaacacccgctcgcgggtgggcctacttcacctatcctgcccggctgacgccgttggatacaccaaggaaagtctacacgaaccctttggcaaaatcctgtatatcgtgcgaaaaaggatggatataccgaaaaaatcgctataatgaccccgaagcagggttatgcagcggaaaagcgctgcttccctgctgttttgtggaatatctaccgactggaaacaggcaaatgcaggaaattactgaactgaggggacaggcgagaggagatcttgatctaatgattcaaacccttgtgaacttctttagaacaaaagaggttcgtaacaagattttcttcacactagcaatgttagtaatttttaaaatagggacttatataccagctccaggagtaaatcctgcagcttttgataatccccaaggttctcaaggtgccactgagttattaaatacttttggtggcggagccttgaaacgattttctatttttgcaatgggtattgtaccctacatcactgcatcaatcgtaatgcaattattacaaatggatattgtccctaaattctcagaatgggcaaaacaaggtgaagtaggtagaagaaagttaaataacgttactcgttatttagcaatttctttagcatttatccaatctataggtatggcattccaatttaataattatctcaaaggtgcgctgattatcaatcagtcaattatgagttatttattaatagcactagttttgacagcaggaactgctttcttaatatggcttggtgatcaaatcactcagttcggtgttggtaatggtatttctattatcatattcccatcaagcttattttaattatactctatcaatgatagagtgtcaatattttttttagtttttcatgaactcgaggggatccaaataaaaaactagtttgacaaataactctatcaatgatagagtgtcaacaaaaaggaggaattaatgatgtctagattagataaaagtaaagtgattaacagcgcattagagctgcttaatgaggtcggaatcgaaggtttaacaacccgtaaactcgcccagaagctaggtgtagagcagcctacattgtattggcatgtaaaaaataagcgggctttgctcgacgccttagccattgagatgttagataggcaccatactcacttttgccctttagaaggggaaagctggcaagattttttacgtaataacgctaaaagttttagatgtgctttactaagtcatcgcgatggagcaaaagtacatttaggtacacggcctacagaaaaacagtatgaaactctcgaaaatcaattagcctttttatgccaacaaggtttttcactagagaatgcattatatgcactcagcgctgtggggcattttactttaggttgcgtattggaagatcaagagcatcaagtcgctaaagaagaaagggaaacacctactactgatagtatgccgccattattacgacaagctatcgaattatttgatcaccaaggtgcagagccagccttcttattcggccttgaattgatcatatgcggattagaaaaacaacttaaatgtgaaagtgggtcttaaaagcagcataacctttttccgtgatggtaacttca

SEQ ID NO: 132 - DNA, 303 bp, Artificial Sequence
  Promoter; promoter leuA
atttttagacaattctaactattaaagtgatatataccattcacggaaggagtataataaaatgcttaatcaatatactgaacatcaaccgacaacttcaaatattattattttattatactctttaggactcgaacgttagtaaatatttactaaacgctttaagtcctatttctgtttgaatgggacttgtaaacgtcccaataatattgggacgtttttttatgttttatctttcaattacttatttttattactataaaacatgattaatcattaaaatttacgggggaatttactatg

SEQ ID NO: 133 - DNA, 303 bp, Artificial Sequence
  Promoter; promoter hlgA2
acttcaaattttcacaaactattgcgaaatccattcctcttccactacaagcaccataattaaacaacaattcaatagaataagacttgcaaaacatagttatgtcgctatataaacgcctgcgaccaataaatcttttaaacataacataatgcaaaaacatcatttaacaatgctaaaaatgtctcttcaatacatgttgatagtaattaacttttaacgaacagttaattcgaaaacgcttacaaatggattattatatatatgaacttaaaattaaatagaaagaaagtgatttctatg

SEQ ID NO: 134 - DNA, 71 bp, Artificial Sequence
  Promoter; promoter hrtAB
gttcatattgagttcatatttcaaccttatactgacgctaaagaagaaatagggagaagtgaatcgatatg

SEQ ID NO: 135 - DNA, 80 bp, Artificial Sequence
  Promoter; promoter hlb
ttcaggctatcaataatgctttgaaatcagcctgtagagtcaataatataccaattattacatcgcacgcattaagacac

SEQ ID NO: 136 - DNA, 80 bp, Artificial Sequence
  Promoter; promoter sbnC
actcattgttcttatttactagcaaaaggtgtatctatacattacatttctaaaagattaggtcataaaaatatagcaat

SEQ ID NO: 137 - DNA, 80 bp, Artificial Sequence
  Promoter; promoter isdI
aactacatccgtgtattcgcatttgttagaagaaaaatttaatgaagaggacaaaaaaacaactaaaattttagaaagta

SEQ ID NO: 138 - DNA, 64 bp, Artificial Sequence
  Promoter; promoter isdG
tgtaatttagggacccattagggactccaaacccaataaatactgttgttacaaggtttctatg

SEQ ID NO: 139 - DNA, 303 bp, Artificial Sequence
  Promoter; promoter sbnE
gaatacttcaaggattaacatatagtgcattgattcaaagtgtcatgtttgttgtcgtgaatgcgtgtcatcaacaacttaaaggcacatttgttggaacgacgaacagtatgttagttgttggtcaaattattggcagtcttagtggcgctgccattacaagttatactacaccagctactacgtttatcgttatgggcgtagtatttgcagtaagtagtttatttttaatttgttcaaccatcactaatcaaatcaacgatcacacattaatgaaattatgggagttgaaacaaaaaagtg

SEQ ID NO: 140 - DNA, 303 bp, Artificial Sequence
  Promoter; promoter lrgA
atgaaaaacgattgaatcccacttattttatacgtattcatcgttcatatattattaacacgaaacacattaaagaagtgcaacaatggtttaactacacttatatggtaatattgacaaatggtgtcaagatgcaagttggacgttcatttatgaaagattttaaagcgtcgataggattactttaacagtaatccttttttttatgcattttacctatgatattttgtatttcggactaaaaatcacgcaaatcgaagtgagccatctatactttagttaaatcaaacgtaggaggcaatg

SEQ ID NO: 141 - DNA, 303 bp, Artificial Sequence
  Promoter; promoter lrgB
gtttagtattattatttgtattattatgtactggtgctgttaagttaggcgaagtcgaaaaagtaggaacgacactaacaaataacattggcttactcttcgtaccagccggtatctcagttgttaactctttaggtgtcattagccaagcaccatttttaatcattggactaataatcgtctcaacaatactattacttatttgtactggctatgtcacacaaattattatgaaagttacttcgagatctaaaggtgacaaagtcacaaaaaagatcaaaatagaggaggcacaagctcatg

SEQ ID NO: 142 - DNA, 303 bp, Artificial Sequence
  Promoter; promoter hlgB
aagatcctagagattatttcgttccagacagtgagttacctcctcttgtacaaagtggatttaacccttcatttatcgccacagtatctcatgaaaaaggttcaagcgatacaagcgaatttgaaattacttacggaagaaacatggatgtcactcatgccattaaaagatcaacgcattatggcaacagttatttagacggacatagagtccataatgcattcgtaaatagaaactatactgttaaatacgaggtcaattggaagactcatgaaatcaaggtgaaaggacagaattgatatg

SEQ ID NO: 143 - DNA, 303 bp, Artificial Sequence
  Promoter; promoter fhuB
tcaaaatgtaacaatgatcagaggcatatgtttaattattgctatgattctagcaggtattgcagttgctatcgctggacaagttgcatttgtaggtttgatggtacctcatatagcaagatttttaattggaactgattatgctaaaattctaccattaacagccttgttaggtgggatactcgtgcttgttgccgatgtgatagcacgatatttaggagaagcgcctgttggtgcaatcatttcatttatcggtgttccttactttttatatttagttaaaaaaggaggacgctcaatatg

SEQ ID NO: 144 - DNA, 303 bp, Artificial Sequence
  Promoter; promoter splF
gttcacctatattaaatagtaagcgagaagcaattggtgttatgtatgctagtgataaaccaacaggtgaaagtacaaggtcatttgctgtttatttctctcctgaaattaagaaatttattgcagataatttagataaataaatcatccatccatacattgataaatgatttttagaaattaacaacaaaatcaacaattttaaacatctctgtgattctatttattcgaaatgatttaaaaaataaaacttcaaaaacctaaccttatatttatacgaatacttagaggagcacaaaaatg

SEQ ID NO: 145 - DNA, 303 bp, Artificial Sequence
  Promoter; promoter SAUSA300_2268
gatgatgtatgtttcgaatttatcaattaacatgtgaggacctcccgaggaatacatggcattaaatacacgtttaatatttataaaggtgacttaattttgttcaagttgattttaccacgctttttttctttattcactaagacttttgaatgaagtttaaaataattgtttatcagtgataaaatatttgcaataagaagagaatggctaaataatcttaattttcagaaaagtaattgtaaccttactggtcttatggtaatatttttcaatattatcgacgaggatgtgttaacaatg

SEQ ID NO: 146 - DNA, 303 bp, Artificial Sequence
  Promoter; promoter SAUSA300_2616
ctatcattataatgagataatgtcatttttaattgagctaaacagacagggaaagacgattattatgattacgcatgatatgcatttattgtctgagtatagttcaagaacagttgtattatcaaaaggacaagtcgttgctgataccacgccagtattgatattaaatgataaaaaaatctgtgagattgcatcattgagacaaacatcgctatttgaaatggccgaatatatagggattagcgagccacagaaattagtacaattatttattaaccatgataggaaggtgagacgccaatg

SEQ ID NO: 147 - DNA, 303 bp, Artificial Sequence
  Promoter; promoter SAUSA300_2617
caggcctattttctaggaaatcgatgatttattttaatatcggtcaaattattgcgaatattatttgctgggcacttattgcaccaacattagatattttgatttataacgaaccggctaacaaggtttatacacaaggtgttatctctgcagtattaaatattatttcagttggtattattgggacaatattattaaaagcatatgcttcatctcaaataaaaaaaggtagtttacgtaaagaataatcattttgttgaatcagatatgtaaatgaatgtagaaaggtaatgatatatcatg

SEQ ID NO: 148 - DNA, 303 bp, Artificial Sequence; identical to SEQ ID NO: 121
  Promoter; promoter isdA

SEQ ID NO: 149 - DNA, 303 bp, Artificial Sequence
  Promoter; promoter isdB
cttcagttgataactttattagcacagttgccttcgcaacacttgcccttttaggttcattatctttattacttttcaaaagaaaagaatctaaataaatcatcgtcacactcataacttaatatattttttattttaaattttatttaacctatgtcatagatatttcataatctataacataggttatttttttataaaataatgttgcaattaactaccatttcaatgtacaatacaagtaatcaattgataatgattatcagttgataatatacaattaggagttgtttctacaacatg

SEQ ID NO: 150 - DNA, 303 bp, Artificial Sequence
  Promoter; promoter fhuA/C
ctttcttgcagatgaataaataaatggtatgagcacacatacttaaatagaagtccacggacaagtttttgaactatgaagacttatctgtgggcgttttttattttataaaagtaatatacaagacatgacaaatcgagctatccaatttaaaaagtaatgttagtcaataagattgaaaaatgttataatgatgttcatgataatcattatcaattgggatgcctttgaaaattgataatttaaaaatagaaattattttttataaacagaaagaattttattgaaagtagggaaattatg

SEQ ID NO: 151 - DNA, 303 bp, Artificial Sequence
  Promoter; promoter ear
tgacacctgctaattcaaacattatttgagacattcttttcaaattaattataaatttttacctatagactagtttgatatttatctacatctcaaaattctcatcaacaatctttcacatccaacatttttactttagtttttataattcaaaacaacaaaacgatgttaaaaaattattctattttttagttaatagatagttaatacatttttgatatttagttaattgttcttttaaaaaaatattattatattttcattgtaaacgtttacaatataaaaaaaggagcaattaaaatg

SEQ ID NO: 152 - DNA, 303 bp, Artificial Sequence
  Promoter; promoter fnb
tgtacaggcgataattatgaaacacttagtatattgttttaaattagataatgatgaatttaatttgaaaaataagtataaaaaatacaagccttgtgtgacaagggtttatgatgacttgaatacaatttataggtatatttcaaataataaaattatcaattaacataaaattaatgacaatcttaacttttcattaactcgcttttttgtattgcttttaaaaaccgaacaatatagacttgcatttattaagtttaaaaaaattaatgaattttgcatttaaagggagatattatagtg

SEQ ID NO: 153 - DNA, 303 bp, Artificial Sequence
  Promoter; promoter splD
attttaaattttgatgcatacattgaacccgggaattcaggatcaccagttctaaattctaacaatgaggtcataggtgtggtgtatggcggtattggaaaaattggttctgaatataatggtgccgtatactttacgcctcaaatcaaagattttattcaaaagcacattgaacaataaacaaatttaaatatacaccatgagcatgtgttcaataattttaatgaaaaacatcggtcgaatataacataaaaaaacgtctatatcaaaagcatcatgaataaacagaggagcacaaaaatg

SEQ ID NO: 154 - DNA, 303 bp, Artificial Sequence
  Promoter; promoter dps
ataatagaaatagaatgtggaaaacaacatggcaccaaccaaatgattatgaaaaatcgttctttttagatgataatgcgaaagtaaaacttactgattgataaaacatacttgctaattgataatggatatactagatgatgaattaaaatttagacatttaaaaagcggaacaccttacatttagattagaataattataaaaaagagagtaaaaacactttacagattagaatcattataatataataattaatataaacaagcaagacgtagacaattttaaggagtgtattaaatatg

SEQ ID NO: 155 - DNA, 300 bp, Artificial Sequence
  Promoter; promoter CH52_00360
gaattctttatagcgcgtgcaatcacaccacaagataaaagattaaaaagtgacaaagcatttattgcatttttagaagaaaccttcgatcagttcttaccattttattctgcataaataactttgtttaaataatagagcacgtaatcacatccatgatttcgtgctcttttttcttaatattaaatcgaacgttcaacataataattcatacttttaaaaaaattaaaataaatttaggttgacctaaacattttattaggttattatattgtccataagaagtagaggtgagtcaaa

SEQ ID NO: 156 - DNA, 303 bp, Artificial Sequence
  Promoter; promoter CH52_00305
cataatccccctccttaaatttgttcatataagattatgatatcttagattgcataaaaagactaggtttaataaaattaaaatgtgacaaattaacgacaagagaaaatgtcaattttgtgacacaaataacatttaatttattgctataatgtatatgttagaaaattttaataagtagaatcatgcatctaaaagagattaatatttaagcttcaaatttgagtaaacgtggattacataattatcccaataaaaaaatcattacgattaagttctttttatgtcgtccacatacaatac

SEQ ID NO: 157 - DNA, 303 bp, Artificial Sequence
  Promoter; promoter CH52_01670
cattttatattccctccgtaaaatataaagttttcttaactagtttataataattttaatttgtagtcaaaaagactttgtaataatgcgttcagttaattataacttacttataccttaatataaacaacttaaaccctttttattatttttaataactctaaagtacaactctaatccgctctctttaaaaatataaatgataataagtgcacataatttctcaatggattttatgaatttaaaatatgttatcatttcactaggacatttgtaatatggtatgatgctatttatgatttt

SEQ ID NO: 158 - DNA, 302 bp, Artificial Sequence
  Promoter; promoter srtB
cataaaaatcctcttttattaacgacgtttcttcagtcatcactaaaccagttgttgtaccgttttagattcgatttcgttgactttgacaaattaagtaaattagcattggaccaccgacaatcattaaaatagcattggctggaatttctaaaggaggctgtatcactcgtcctaataaatcagccactaacaatagccatgcaccaataactgtagaaaacggaataagtactctgtaattgcccccaactagctttctaaccacatgtggcacaataatacctaaaaaggctagttgt

SEQ ID NO: 159 - DNA, 303 bp, Artificial Sequence
  Promoter; promoter sbnA
caaaagcgcttcctcctcaaatttaaaattctataatattgtgtgttacctaattgataatgattctcactatcaagtaattaggattatattttttatgcatttatatgtcaaataattataagttgcatgtaaatcataaatattttattgacttaggaaaaaatttaattcatactaaatcgtgataatgattctcattgtcatacatcacgaaggaggctaattagtcaatgaataaagtaattaaaatgcttgttgttacgcttgctttcctacttgttttagcaggatgtagtggga

SEQ ID NO: 160 - DNA, 303 bp, Artificial Sequence
  Promoter; promoter clfA
cattttattccctctttttaaaaagtcattttatattaactatataccctttaaagatatatttaatctctgttaatggaattatacactaaaattgcattatagcaattaatttgtatcgatattttattatccacaataatactttactaacaaacattttatttattgctattttaagaattacaaacgacaacgtacgatttgattgcaaacattttttattattaatatgaactctacctaatgtaatcctagctttaaatcatattttttcaaaagcagatgtgtaatttatggtac

SEQ ID NO: 161 - DNA, 303 bp, Artificial Sequence
  Promoter; promoter emp homolog
catctgttatttctcctttatatagactcaatattataaccaatataatttccctgttatattcactaacagcattatataccagaattttcagtataataattaacttgaagtaaacgttgtcttaacatttttattgtttttcagcttaaaattaattattgatattgatagttaagcataataattttttcgtaatataaagtgaaaaaagtaatagtccacacctgtttagaatgtggactatactagattgcatcattgaaatgatgactttgatattatttattgctagtttaaaat

SEQ ID NO: 162 - DNA, 283 bp, Artificial Sequence
  Promoter; promoter rsaC
cacgctgtgttttaatgaagtaagatgaattgatgttgatgcaacctaaaatattggtatctccaatattttaggctacacatcaacataacaaagtcgaaggctaatagtcccatatcgtgcgttaaatatatattaccctcctattaatatatataccgttcccgatcgcacgatatggtggtattagaacttctctttgaacgaaagagaaaagctagaacttatgcagttttaattaaactgtaaacatttgtcactctttaaatcaaagagtaaagtt

SEQ ID NO: 163 - DNA, 303 bp, Artificial Sequence
  Promoter; promoter hlgA1
aacaatttgtattttacaaacattaattaaaaataaaagcaagacattcgtgcaatcggttaccttaaattgtttacaactgtcaacaataccaaggttttattaactatatttctcacaaaattagcttttagcattccaaacaaaaaaggttaaattgaacggaattatggcatttttaacttaattgtaaaaaagttgataatggtcaattgttaatgaacagttaattataataacgtccaaaatatattattatttaattaagttaaataaaattatagaaagaaagtgaaacttatg

SEQ ID NO: 164 - DNA, 30 bp, Artificial Sequence
  Primer; forward primer isdA
tatatgcatgcctatctgcggcatttgcag

SEQ ID NO: 165 - DNA, 32 bp, Artificial Sequence
  Primer; reverse primer isdA
gatacctgcaggttgttttcctcctaaggata

SEQ ID NO: 166 - DNA, 32 bp, Artificial Sequence
  Primer; forward primer isdB
gatgcgcatgccttcagttgataactttatta

SEQ ID NO: 167 - DNA, 32 bp, Artificial Sequence
  Primer; reverse primer isdB
gatgcctgcaggttgtagaaacaactcctaat

SEQ ID NO: 168 - DNA, 32 bp, Artificial Sequence
  Primer; forward primer isdI
gatacgcatgcttactcgtagcagttttttgt

SEQ ID NO: 169 - DNA, 32 bp, Artificial Sequence
  Primer; reverse primer isdI
gatagctgcaggggcaatcactcctctatttt

SEQ ID NO: 170 - DNA, 32 bp, Artificial Sequence
  Primer; forward primer isdG
gatgcgcatgcaaacacaagataattgaattt

SEQ ID NO: 171 - DNA, 33 bp, Artificial Sequence
  Primer; reverse primer isdG
gatgcctgcagaattatcctcttttctgtttaa

SEQ ID NO: 172 - DNA, 36 bp, Artificial Sequence
  Primer; forward primer sbnC
gaatcgcatgcctttattaaagctgacaaagtcgta

SEQ ID NO: 173 - DNA, 32 bp, Artificial Sequence
  Primer; reverse primer sbnC
gaaatcctgcagtgttcagacacctcgcattc

SEQ ID NO: 174 - DNA, 51 bp, Artificial Sequence
  Primer; forward primer sbnE
taactgactaggcggccgcgaatacttcaaggattaacatatagtgcattg

SEQ ID NO: 175 - DNA, 62 bp, Artificial Sequence
  Primer; reverse primer sbnE
ccagtgaaaagttcttctcctttactcatttttttgtttcaactcccataatttcattaatg

SEQ ID NO: 176 - DNA, 53 bp, Artificial Sequence
  Primer; forward primer lrgA
taactgactaggcggccgcatgaaaaacgattgaatcccacttattttatacg

SEQ ID NO: 177 - DNA, 56 bp, Artificial Sequence
  Primer; reverse primer lrgA
ccagtgaaaagttcttctcctttactcattgcctcctacgtttgatttaactaaag

SEQ ID NO: 178 - DNA, 58 bp, Artificial Sequence
  Primer; forward primer lrgB
taactgactaggcggccgcgtttagtattattatttgtattattatgtactggtgctg

SEQ ID NO: 179 - DNA, 52 bp, Artificial Sequence
  Primer; reverse primer lrgB
ccagtgaaaagttcttctcctttactcatgagcttgtgcctcctctattttg

SEQ ID NO: 180 - DNA, 46 bp, Artificial Sequence
  Primer; forward primer hlgB
taactgactaggcggccgcaagatcctagagattatttcgttccag

SEQ ID NO: 181 - DNA, 57 bp, Artificial Sequence
  Primer; reverse primer hlgB
ccagtgaaaagttcttctcctttactcatatcaattctgtcctttcaccttgatttc

SEQ ID NO: 182 - DNA, 53 bp, Artificial Sequence
  Primer; forward primer fhuA
taactgactaggcggccgcctttcttgcagatgaataaataaatggtatgagc

SEQ ID NO: 183 - DNA, 60 bp, Artificial Sequence
  Primer; reverse primer fhuA
ccagtgaaaagttcttctcctttactcataatttccctactttcaataaaattctttctg

SEQ ID NO: 184 - DNA, 44 bp, Artificial Sequence
  Primer; forward primer fhuB
taactgactaggcggccgctcaaaatgtaacaatgatcagaggc

SEQ ID NO: 185 - DNA, 65 bp, Artificial Sequence
  Primer; reverse primer fhuB
ccagtgaaaagttcttctcctttactcatattgagcgtcctccttttttaactaaatataaaaag

SEQ ID NO: 186 - DNA, 47 bp, Artificial Sequence
  Primer; forward primer ear
taactgactaggcggccgctgacacctgctaattcaaacattatttg

SEQ ID NO: 187 - DNA, 65 bp, Artificial Sequence
  Primer; reverse primer ear
ccagtgaaaagttcttctcctttactcattttaattgctcctttttttatattgtaaacgtttac

SEQ ID NO: 188 - DNA, 48 bp, Artificial Sequence
  Primer; forward primer fnb
taactgactaggcggccgctgtacaggcgataattatgaaacacttag

SEQ ID NO: 189 - DNA, 74 bp, Artificial Sequence
  Primer; reverse primer fnb
ccagtgaaaagttcttctcctttactcattataatatctccctttaaatgcaaaattcattaatttttttaaac

SEQ ID NO: 190 - DNA, 47 bp, Artificial Sequence
  Primer; forward primer hlb
taactgactaggcggccgcttcaggctatcaataatgctttgaaatc

SEQ ID NO: 191 - DNA, 59 bp, Artificial Sequence
  Primer; reverse primer hlb
ccagtgaaaagttcttctcctttactcatagaaaccttgtaacaacagtatttattggg

SEQ ID NO: 192 - DNA, 50 bp, Artificial Sequence
  Primer; forward primer splF
taactgactaggcggccgcgttcacctatattaaatagtaagcgagaagc

SEQ ID NO: 193 - DNA, 65 bp, Artificial Sequence
  Primer; reverse primer splF
ccagtgaaaagttcttctcctttactcatttttgtgctcctctaagtattcgtataaatataagg

SEQ ID NO: 194 - DNA, 51 bp, Artificial Sequence
  Primer; forward primer splD
taactgactaggcggccgcattttaaattttgatgcatacattgaacccgg

SEQ ID NO: 195 - DNA, 58 bp, Artificial Sequence
  Primer; reverse primer splD
ccagtgaaaagttcttctcctttactcatttttgtgctcctctgtttattcatgatgc

SEQ ID NO: 196 - DNA, 52 bp, Artificial Sequence
  Primer; forward primer dps
taactgactaggcggccgcataatagaaatagaatgtggaaaacaacatggc

SEQ ID NO: 197 - DNA, 60 bp, Artificial Sequence
  Primer; reverse primer dps
ccagtgaaaagttcttctcctttactcatatttaatacactccttaaaattgtctacgtc

SEQ ID NO: 198 - DNA, 55 bp, Artificial Sequence
  Primer; forward primer SAUSA 300_2268
taactgactaggcggccgcgatgatgtatgtttcgaatttatcaattaacatgtg

SEQ ID NO: 199 - DNA, 57 bp, Artificial Sequence
  Primer; reverse primer SAUSA 300_2268
ccagtgaaaagttcttctcctttactcattgttaacacatcctcgtcgataatattg

SEQ ID NO: 200 - DNA, 57 bp, Artificial Sequence
  Primer; forward primer SAUSA 300_2616
taactgactaggcggccgcctatcattataatgagataatgtcatttttaattgagc

SEQ ID NO: 201 - DNA, 49 bp, Artificial Sequence
  Primer; reverse primer SAUSA 300_2616
ccagtgaaaagttcttctcctttactcattggcgtctcaccttcctatc

SEQ ID NO: 202 - DNA, 45 bp, Artificial Sequence
  Primer; forward primer SAUSA 300_2617
taactgactaggcggccgccaggcctattttctaggaaatcgatg

SEQ ID NO: 203 - DNA, 65 bp, Artificial Sequence
  Primer; reverse primer SAUSA 300_2617
ccagtgaaaagttcttctcctttactcatgatatatcattacctttctacattcatttacatatc

SEQ ID NO: 204 - DNA, 60 bp, Artificial Sequence
  Primer; forward primer hlgA2
cgttaactaattaatttaagaaggagatatacatacttcaaattttcacaaactattgcg

SEQ ID NO: 205 - DNA, 70 bp, Artificial Sequence
  Primer; reverse primer hlgA2
ccagtgaaaagttcttctcctttactcatagaaatcactttctttctatttaattttaagttcatatata

SEQ ID NO: 206 - DNA, 60 bp, Artificial Sequence
  Primer; forward primer hrtAB
cgttaactaattaatttaagaaggagatatacatgttcatattgagttcatatttcaacc

SEQ ID NO: 207 - DNA, 55 bp, Artificial Sequence
  Primer; reverse primer hrtAB
ccagtgaaaagttcttctcctttactcatatcgattcacttctccctatttcttc

SEQ ID NO: 208 - DNA, 29 bp, Artificial Sequence
  Primer; forward primer for pCN56 plasmid with hlgA2, hrtAB promoters
atgagtaaaggagaagaacttttcactgg

SEQ ID NO: 209 - DNA, 40 bp, Artificial Sequence
  Primer; reverse primer for pCN56 plasmid with hlgA2, hrtAB promoters
atgtatatctccttcttaaattaattagttaacgaattcg

SEQ ID NO: 210 - DNA, 29 bp, Artificial Sequence
  Primer; forward primer for pCN56 plasmid
atgagtaaaggagaagaacttttcactgg

SEQ ID NO: 211 - DNA, 39 bp, Artificial Sequence
  Primer; reverse primer for pCN56 plasmid
gcggccgcctagtcagttaactcaaaggcggtaatacgg

SEQ ID NO: 212 - DNA, 20 bp, Artificial Sequence
  Primer; forward qRT PCR primer for gyrB housekeeping
ttggtacaggaatcggtggc

SEQ ID NO: 213 - DNA, 20 bp, Artificial Sequence
  Primer; reverse qRT PCR primer for gyrB housekeeping
tccatccacatcggcatcag

SEQ ID NO: 214 - DNA, 20 bp, Artificial Sequence
  Primer; isdA forward qRT PCR primer
gcaacagaagctacgaacgc

SEQ ID NO: 215 - DNA, 22 bp, Artificial Sequence
  Primer; isdA reverse qRT PCR primer
agagccatctttttgcacttgg

SEQ ID NO: 216 - DNA, 25 bp, Artificial Sequence
  Primer; isdB forward qRT PCR primer
gcaacaattttatcattatgccagc

SEQ ID NO: 217 - DNA, 22 bp, Artificial Sequence
  Primer; isdB reverse qRT PCR primer
tggcaactttttgtcaccttca

SEQ ID NO: 218 - DNA, 21 bp, Artificial Sequence
  Primer; isdI forward qRT PCR primer
accgaggatacagacgaagtt

SEQ ID NO: 219 - DNA, 21 bp, Artificial Sequence
  Primer; isdI reverse qRT PCR primer
tgctgtccatcgtcatcactt

SEQ ID NO: 220 - DNA, 21 bp, Artificial Sequence
  Primer; isdG forward primer
aaccaatccgtaaaagcttgc

SEQ ID NO: 221 - DNA, 20 bp, Artificial Sequence
  Primer; isdG reverse qRT PCR primer
aggctttgatggcatgtttg

SEQ ID NO: 222 - DNA, 21 bp, Artificial Sequence
  Primer; sbnC forward qRT PCR primer
agggaagggtgtctaagcaac

SEQ ID NO: 223 - DNA, 20 bp, Artificial Sequence
  Primer; sbnC reverse qRT PCR primer
tcagtccttcttcaacgcga

SEQ ID NO: 224 - DNA, 20 bp, Artificial Sequence
  Primer; sbnE forward qRT PCR primer
attcgctttagccgcaatgg

SEQ ID NO: 225 - DNA, 20 bp, Artificial Sequence
  Primer; sbnE reverse qRT PCR primer
gcaacttgtagcgcatcgtc

SEQ ID NO: 226 - DNA, 21 bp, Artificial Sequence
  Primer; lrgA forward qRT PCR primer
gataccggctggtacgaagag

SEQ ID NO: 227 - DNA, 21 bp, Artificial Sequence
  Primer; lrgA reverse qRT PCR primer
tggtgctgttaagttaggcga

SEQ ID NO: 228 - DNA, 20 bp, Artificial Sequence
  Primer; lrgB forward qRT PCR primer
acaaagacaggcacaactgc

SEQ ID NO: 229 - DNA, 20 bp, Artificial Sequence
  Primer; lrgB reverse qRT PCR primer
ggtgtagcaccagccaaaga

SEQ ID NO: 230 - DNA, 21 bp, Artificial Sequence
  Primer; hlgB forward qRT PCR primer
tggttggggaccttatggaag

SEQ ID NO: 231 - DNA, 20 bp, Artificial Sequence
  Primer; hlgB reverse qRT PCR primer
ggcatttggtgttgcgctat

SEQ ID NO: 232 - DNA, 21 bp, Artificial Sequence
  Primer; fhuA forward qRT PCR primer
cacgttgtctttgaccaccac

SEQ ID NO: 233 - DNA, 21 bp, Artificial Sequence
  Primer; fhuA reverse qRT PCR primer
tgggcaatggaagttacagga

SEQ ID NO: 234 - DNA, 20 bp, Artificial Sequence
  Primer; fhuB forward qRT PCR primer
caatacctgctggaacccca

SEQ ID NO: 235 - DNA, 20 bp, Artificial Sequence
  Primer; fhuB reverse qRT PCR primer
gggtccgcatattgccaaac

SEQ ID NO: 236 - DNA, 21 bp, Artificial Sequence
  Primer; ear forward qRT PCR primer
ccacttgtcagatctgctcct

SEQ ID NO: 237 - DNA, 24 bp, Artificial Sequence
  Primer; ear reverse qRT PCR primer
ggtttggttacagatggacaaaca

SEQ ID NO: 238 - DNA, 19 bp, Artificial Sequence
  Primer; fnb forward qRT PCR primer
cgcagtgagcgaccataca

SEQ ID NO: 239 - DNA, 20 bp, Artificial Sequence
  Primer; fnb reverse qRT PCR primer
ttggtccttgtgcttgacca

SEQ ID NO: 240 - DNA, 20 bp, Artificial Sequence
  Primer; hlb forward qRT PCR primer
ctacgccaccatcttcagca

SEQ ID NO: 241 - DNA, 20 bp, Artificial Sequence
  Primer; hlb reverse qRT PCR primer
acacctgtactcggtcgttc

SEQ ID NO: 242 - DNA, 22 bp, Artificial Sequence
  Primer; splF forward qRT PCR primer
tgcaattattcagcctggtagc

SEQ ID NO: 243 - DNA, 22 bp, Artificial Sequence
  Primer; splF reverse qRT PCR primer
cctgatggcttattaccggcat

SEQ ID NO: 244 - DNA, 20 bp, Artificial Sequence
  Primer; splD forward qRT PCR primer
agtgacatctgatgcggttg

SEQ ID NO: 245 - DNA, 21 bp, Artificial Sequence
  Primer; splD reverse qRT PCR primer
aacaccaattgcttctcgctt

SEQ ID NO: 246 - DNA, 20 bp, Artificial Sequence
  Primer; dps forward qRT PCR primer
agcggtaggaggaaaccctg

SEQ ID NO: 247 - DNA, 22 bp, Artificial Sequence
  Primer; dps reverse qRT PCR primer
gttctgcagagtaacctttcgc

SEQ ID NO: 248 - DNA, 21 bp, Artificial Sequence
  Primer; srtB  forward qRT PCR primer
tgagcgagaacatcgacgtaa

SEQ ID NO: 249 - DNA, 20 bp, Artificial Sequence
  Primer; srtB reverse qRT PCR primer
ccgacatggtgcccgtataa

SEQ ID NO: 250 - DNA, 21 bp, Artificial Sequence
  Primer; emp  forward qRT PCR primer
tcgcgtgaatgtagcaacaaa

SEQ ID NO: 251 - DNA, 21 bp, Artificial Sequence
  Primer; emp  reverse qRT PCR primer
acttctgggcctttagcaaca

SEQ ID NO: 252 - DNA, 20 bp, Artificial Sequence
  Primer; sbnA  forward qRT PCR primer
cctggaggcagcatgaaaga

SEQ ID NO: 253 - DNA, 20 bp, Artificial Sequence
  Primer; sbnA  reverse qRT PCR primer
cattgccaacgcaatgccta

SEQ ID NO: 254 - DNA, 20 bp, Artificial Sequence
  Primer; CH52_360 forward qRT PCR primer
ttcaactcgaacgctgacga

SEQ ID NO: 255 - DNA, 20 bp, Artificial Sequence
  Primer; CH52_360 reverse qRT PCR primer
ttgcacccattgttgcacct

SEQ ID NO: 256 - DNA, 20 bp, Artificial Sequence
  Primer; CH52_305 forward qRT PCR primer
ttcctggagcagtaccacca

SEQ ID NO: 257 - DNA, 22 bp, Artificial Sequence
  Primer; CH52_305 reverse qRT PCR primer
cagcgcaatcgctgttaaacta

SEQ ID NO: 258 - DNA, 20 bp, Artificial Sequence
  Primer; CH521670 forward qRT PCR primer
gcgattatgggaccaaacgg

SEQ ID NO: 259 - DNA, 21 bp, Artificial Sequence
  Primer; CH521670 reverse qRT PCR primer
acttcatagcttgggtgtccc

SEQ ID NO: 260 - DNA, 20 bp, Artificial Sequence
  Primer; clfA  forward qRT PCR primer
tccagcacaacaggaaacga

SEQ ID NO: 261 - DNA, 20 bp, Artificial Sequence
  Primer; clfA  reverse qRT PCR primer
tagcttcaccagttaccggc

SEQ ID NO: 262 - DNA, 20 bp, Artificial Sequence
  Primer; SAUSA300_2268 forward qRT PCR primer
gcttctacagctttgccgat

SEQ ID NO: 263 - DNA, 21 bp, Artificial Sequence
  Primer; SAUSA300_2268 reverse qRT PCR primer
gatttggtgcttactgccacc

SEQ ID NO: 264 - DNA, 20 bp, Artificial Sequence
  Primer; SAUSA300_2616 forward qRT PCR primer
acaagcgcaacaagcaagag

SEQ ID NO: 265 - DNA, 23 bp, Artificial Sequence
  Primer; SAUSA300_2616 reverse qRT PCR primer
tgcgtttgatacctttaacacgg

SEQ ID NO: 266 - DNA, 21 bp, Artificial Sequence
  Primer; SAUSA300_2617 forward qRT PCR primer
gggctgaaaaagttggcatga

SEQ ID NO: 267 - DNA, 20 bp, Artificial Sequence
  Primer; SAUSA300_2617 reverse qRT PCR primer
acgcgttgtttttgacctcc

SEQ ID NO: 268 - DNA, 21 bp, Artificial Sequence
  Primer; hlgA2 forward qRT PCR primer
tgatttctgcaccttgaccga

SEQ ID NO: 269 - DNA, 20 bp, Artificial Sequence
  Primer; hlgA2 reverse qRT PCR primer
agcccctttagccaatccat

SEQ ID NO: 270 - DNA, 22 bp, Artificial Sequence
  Primer; hrtAB  forward qRT PCR primer
acacaacaacaacgtgatgagc

SEQ ID NO: 271 - DNA, 20 bp, Artificial Sequence
  Primer; hrtAB  reverse qRT PCR primer
taacggtgcttgctctgctt

SEQ ID NO: 272 - DNA, 204 bp, Staphylococcus aureus
cgcagagaggaggtgtataaggtgatgcttattttcgttcacatcatagcaccagtcatcagtggctgtgccattgcgtttttttcttattggctaagtagacgcaatacaaaataggtgacatatagccgcaccaataaaaatcccctcactaccgcaaatagtgaggggattggtgtataagtaaatacttattttcgttgt

SEQ ID NO: 273 - DNA, 60 bp, Staphylococcus aureus
cccctcactaccgcaaatagtgaggggattggtgtataagtaaatacttattttcgttgt

SEQ ID NO: 274 - DNA, 144 bp, Staphylococcus aureus
cgcagagaggaggtgtataaggtgatgcttattttcgttcacatcatagcaccagtcatcagtggctgtgccattgcgtttttttcttattggctaagtagacgcaatacaaaataggtgacatatagccgcaccaataaaaat

SEQ ID NO: 275 - DNA, 120 bp, Staphylococcus aureus
atgcttattttcgttcacatcatagcaccagtcatcagtggctgtgccattgcgtttttttcttattggctaagtagacgcaatacaaaataggtgacatatagccgcaccaataaaaat

SEQ ID NO: 276 - DNA, 31 bp, Artificial Sequence
  BPC_670 oligo for plasmid construction
gctcagatctgttaacggtaccatcatactc

SEQ ID NO: 277 - DNA, 21 bp, Artificial Sequence
  BPC_671 oligo for plasmid construction
cactggccgtcgttttacaac

SEQ ID NO: 278 - DNA, 55 bp, Artificial Sequence
  BPC_672 oligo for plasmid construction
gagtatgatggtaccgttaacagatctgagccgcagagaggaggtgtataaggtg

SEQ ID NO: 279 - DNA, 60 bp, Artificial Sequence
  BPC_674 oligo for plasmid construction
gagtatgatggtaccgttaacagatctgagcatggtggcattactgaaatctttagaaag

SEQ ID NO: 280 - DNA, 51 bp, Artificial Sequence
  BPC_675 oligo for plasmid construction
gagtatgatggtaccgttaacagatctgagcatggcactgcctaaaacggg

SEQ ID NO: 281 - DNA, 61 bp, Artificial Sequence
  BPC_676 oligo for plasmid construction
gagtatgatggtaccgttaacagatctgagcatggctaatgaaactaaacaacctaaagtt

SEQ ID NO: 282 - DNA, 41 bp, Artificial Sequence
  BPC_677 oligo for plasmid construction
gttgtaaaacgacggccagtgcccgggctcagctattatca

SEQ ID NO: 283 - DNA, 39 bp, Artificial Sequence
  BPC_678 oligo for plasmid construction
gttgtaaaacgacggccagtggcggccgcccatgcatgc

SEQ ID NO: 284 - DNA, 93 bp, Staphylococcus aureus
atgcttattttcgttcacatcatagcaccagtcatcagtggctgtgccattgcgtttttttcttattggctaagtagacgcaatacaaaatag

SEQ ID NO: 285 - protein, 29 aa, Staphylococcus aureus
LIFVHIIAPVISGCAIAFFSYWLSRRNTK

SEQ ID NO: 286 - DNA, 795 bp, Artificial Sequence
  187-lysK toxin gene encodes engineered phage lysin protein from the Staphylococcus aureus phage
atggcactgcctaaaacgggtaaaccaacggcaaaacaggtggttgactgggcaatcaatttaatcggcagtggtgtcgatgttgatggttattatggtcggcaatgttgggatttacctaactatatttttaatagatactggaactttaagacaccaggcaacgcaagagatatggcatggtatagatatcctgaagggtttaaagtgtttagaaacacttctgattttgtccctaaaccaggtgatatagcagtgtggacaggtggtaattacaattggaacacttggggacacactggtattgttgtaggtccatcaactaaaagttacttttatagtgtagatcagaattggaataactctaactcttacgttggtagtcctgcagcaaagataaaacatagttattttggtgtaactcattttgttagacccgcatacaaagcagaaccgaaacctacaccaccactggacagtacaccggcaactagaccagttacaggttcttggaaaaagaaccagtacggaacttggtataaaccggaaaatgcaacatttgtcaatggtaaccaacctatagtaactagaataggttctccattcttaaatgctccagtaggcggtaacttaccggcaggggctacaattgtatatgacgaagtttgtatccaagcaggtcacatttggataggttataatgcttacaacggtaacagagtatattgccctgttagaacttgtcaaggtgttccacctaatcaaatacctggcgttgcctggggagtattcaaa

SEQ ID NO: 287 - protein, 265 aa, Artificial Sequence
  recombinant phage lysin LysK toxin
MALPKTGKPTAKQVVDWAINLIGSGVDVDGYYGRQCWDLPNYIFNRYWNFKTPGNARDMAWYRYPEGFKVFRNTSDFVPKPGDIAVWTGGNYNWNTWGHTGIVVGPSTKSYFYSVDQNWNNSNSYVGSPAAKIKHSYFGVTHFVRPAYKAEPKPTPPLDSTPATRPVTGSWKKNQYGTWYKPENATFVNGNQPIVTRIGSPFLNAPVGGNLPAGATIVYDEVCIQAGHIWIGYNAYNGNRVYCPVRTCQGVPPNQIPGVAWGVFK

SEQ ID NO: 288 - DNA, 504 bp, Staphylococcus aureus
atggctaatgaaactaaacaacctaaagttgttggaggaataaactttagcacaagaactaagagtaaaacattttgggtagcaattatatcagcagtagcagtatttgctaatcaaattacaggtgcttttggtttagactactcagctcaaattgagcaaggtgtaaatatcataggttctatactaacattattagcaggtttaggtattattgttgataataatactaaaggtcttaaagatagtgatattgttcaaacagattatataaaacctcgtgatagtaaagaccctaatgaatttgttcaatggcaagcaaatgcaaacacagctagcactttcgaattagacaactatgaaaacaatgcagaacctgatacagatgatagtgatgaagtacctgctattgaagatgaaattgatggcggttcagcaccttctcaagatgaagaagataccgaggaacacggtaaagtatttgcagaggaggaagttaagtag

SEQ ID NO: 289 - protein, 167 aa, Staphylococcus aureus
MANETKQPKVVGGINFSTRTKSKTFWVAIISAVAVFANQITGAFGLDYSAQIEQGVNIIGSILTLLAGLGIIVDNNTKGLKDSDIVQTDYIKPRDSKDPNEFVQWQANANTASTFELDNYENNAEPDTDDSDEVPAIEDEIDGGSAPSQDEEDTEEHGKVFAEEEVK

SEQ ID NO: 290 - DNA, 135 bp, Staphylococcus aureus
atggtggcattactgaaatctttagaaaggagacgcctaatgattacaattagtaccatgttgcagtttggtttattccttattgcattgataggtctagtaatcaagcttattgaattaagcaataaaaaataa

SEQ ID NO: 291 - protein, 44 aa, Staphylococcus aureus
MVALLKSLERRRLMITISTMLQFGLFLIALIGLVIKLIELSNKK

SEQ ID NO: 292 - DNA, 20 bp, Artificial Sequence
  Primer; gfp primer
ctgtccacacaatctgccct

SEQ ID NO: 293 - DNA, 20 bp, Artificial Sequence
  Primer; gfp primer
tgccatgtgtaatcccagca

SEQ ID NO: 294 - DNA, 25 bp, Artificial Sequence
  Primer; DR_022 primer
caagcttatcgataccgtcgacctc

SEQ ID NO: 295 - DNA, 23 bp, Artificial Sequence
  Primer; DR_023 primer
gggatccactagttctagagcgg

SEQ ID NO: 296 - DNA, 31 bp, Artificial Sequence
  Primerr; DR_237 primer
gcaactggtacatcacaattggtactctcac

SEQ ID NO: 297 - DNA, 32 bp, Artificial Sequence
  Primer; DR_238 primer
gaccacgcatacctatctataaacggacaatg

SEQ ID NO: 298 - DNA, 44 bp, Artificial Sequence
  Primer; DR_255 primer
gtccaattagatggcatgtaactgggcagtgtcttaaaaaatcg

SEQ ID NO: 299 - DNA, 55 bp, Artificial Sequence
  Primer; DR_241 primer
caggccaatttggcatagagccggatgtgctgcaaggcgattaagttgggtaacg

SEQ ID NO: 300 - DNA, 45 bp, Artificial Sequence
  Primer; DR_256 primer
gttacatgccatctaattggacaaattctatgagagtagattttg

SEQ ID NO: 301 - DNA, 33 bp, Artificial Sequence
  Primer; DR_257 primer
gccaaatcgctttcgtgtatacgattcccagtc

SEQ ID NO: 302 - DNA, 30 bp, Artificial Sequence
  Primer; DR_240 primer
ggctctatgccaaattggcctgatgagttc

SEQ ID NO: 303 - DNA, 53 bp, Artificial Sequence
  Primer; DR_236 primer
gctctagaactagtggatcccggcgattttattgtgacaagagactgaagagc

SEQ ID NO: 304 - DNA, 108 bp, Staphylococcus aureus
atgttcaatttattaattaacatcatgacttcagctttaagcggctgtcttgttgcgttttttgcacattggttacgaacgcgcaacaataaaaaaggtgacaaataa

SEQ ID NO: 305 - protein, 35 aa, Staphylococcus aureus
MFNLLINIMTSALSGCLVAFFAHWLRTRNNKKGDK

SEQ ID NO: 306 - DNA, 77 bp, Staphylococcus aureus
tataattaattacataataaattgaacatctaaatacaccaaatcccctcactactgccatagtgaggggatttatt

SEQ ID NO: 307 - DNA, 140 bp, Staphylococcus aureus
atatatagaaaaagggcaacatgcgcaaacatgttaccctaatgagcccgttaaaaagacggtggctattttagattaaagattaaattaataaccatttaaccatcgaaaccagccaaagttagcgatggttatttttt

SEQ ID NO: 308 - DNA, 76 bp, Artificial Sequence
  holin antitoxin gene
tataattgagatagtttcattagctatttacttatacaccaatcccctcactatttgcggtagtgaggggattttt

SEQ ID NO: 309 - DNA, 76 bp, Artificial Sequence
  187-lysK antitoxin gene
tataattgagattttaggcagtgctatttacttatacaccaatcccctcactatttgcggtagtgaggggattttt

SEQ ID NO: 310 - DNA, 140 bp, Artificial Sequence; identical to SEQ ID NO: 307
  sprG antitoxin gene (sprF)

SEQ ID NO: 311 - DNA, 74 bp, Staphylococcus aureus
tataattgagataacgaaaataagtatttacttatacaccaatcccctcactatttgcggtagtgaggggattt

SEQ ID NO: 312 - DNA, 90 bp, Staphylococcus aureus
tataattaattacataataaattgaacatctaaatacaccaaatcccctcactactgccatagtgaggggatttatttaggtgttggtta

SEQ ID NO: 313 - DNA, 158 bp, Staphylococcus aureus
atgattatcactagccctacagaagcgagaaaagatttttatcaattactaaaaaatgttaataataatcacgaaccaatttatattagtggcaataatgccgaaaataatgctgtgattataggtttagaagattggaaaagtatacaagagacaat

SEQ ID NO: 314 - protein, 85 aa, Staphylococcus aureus
MIITSPTEARKDFYQLLKNVNNNHEPIYISGNNAENNAVIIGLEDWKSIQETIYLESTGTMDKVREREKDNSGTTNIDDIDWDNL

SEQ ID NO: 315 - DNA, 159 bp, Staphylococcus aureus
atgagcaattacacggttaagattaaaaattcagcgaaatcagatttaaggaaaataaaacattcttatttaaagaagtcatttttagaaattgttgagactttaaaaaatgatccgtataaaataacacaatcttttgaaaaattagagcctaaatat

SEQ ID NO: 316 - protein, 88 aa, Staphylococcus aureus
MSNYTVKIKNSAKSDLRKIKHSYLKKSFLEIVETLKNDPYKITQSFEKLEPKYLERYSRRINHQHRVVYTVDDRNKEVLILSAWSHYD

SEQ ID NO: 317 - DNA, 738 bp, Staphylococcus simulans
atgacacatgaacattcagcacaatggttgaataattacaaaaaaggatatggttacggtccttatccattaggtataaatggcggtatgcactacggagttgatttttttatgaatattggaacaccagtaaaagctatttcaagcggaaaaatagttgaagctggttggagtaattacggaggaggtaatcaaataggtcttattgaaaatgatggagtgcatagacaatggtatatgcatctaagtaaatataatgttaaagtaggagattatgtcaaagctggtcaaataatcggttggtctggaagcactggttattctacagcaccacatttacacttccaaagaatggttaattcattttcaaattcaactgcccaagatccaatgcctttcttaaagagcgcaggatatggaaaagcaggtggtacagtaactccaacgccgaatacaggttggaaaacaaacaaatatggcacactatataaatcagagtcagctagcttcacacctaatacagatataataacaagaacgactggtccatttagaagcatgccgcagtcaggagtcttaaaagcaggtcaaacaattcattatgatgaagtgatgaaacaagacggtcatgtttgggtaggttatacaggtaacagtggccaacgtatttacttgcctgtaagaacatggaataaatctactaatactttaggtgttctttggggaactataaagtga

SEQ ID NO: 318 - protein, 245 aa, Staphylococcus simulans
MTHEHSAQWLNNYKKGYGYGPYPLGINGGMHYGVDFFMNIGTPVKAISSGKIVEAGWSNYGGGNQIGLIENDGVHRQWYMHLSKYNVKVGDYVKAGQIIGWSGSTGYSTAPHLHFQRMVNSFSNSTAQDPMPFLKSAGYGKAGGTVTPTPNTGWKTNKYGTLYKSESASFTPNTDIITRTTGPFRSMPQSGVLKAGQTIHYDEVMKQDGHVWVGYTGNSGQRIYLPVRTWNKSTNTLGVLWGTIK

SEQ ID NO: 319 - DNA, 76 bp, Artificial Sequence
  proposed lysostaphin antitoxin gene; encodes RNA antitoxin for lysostaphin
tataattgagatatgttcatgtgttatttacttatacaccaatcccctcactatttgcggtagtgaggggattttt

SEQ ID NO: 320 - DNA, 157 bp, Staphylococcus aureus
atgattagacgaggagatgtttatttagcagatttatcaccagtacagggatctgaacaagggggagtcagacctgtagtcataattcaaaatgatactggtaataaatatagtcctacagttattgttgcggcaataactggtaggattaataaag

SEQ ID NO: 321 - protein, 120 aa, Staphylococcus aureus
MIRRGDVYLADLSPVQGSEQGGVRPVVIIQNDTGNKYSPTVIVAAITGRINKAKIPTHVEIEKKKYKLDKDSVILLEQIRTLDKKRLKEKLTYLSDDKMKEVDNALMISLGLNAVAHQKN

SEQ ID NO: 322 - DNA, 158 bp, Staphylococcus aureus
atgttatcttttagtcaaaatagaagtcatagcttagaacaatctttaaaagaaggatattcacaaatggctgatttaaatctctccctagcgaacgaagcttttccgatagagtgtgaagcatgcgattgcaacgaaacatatttatcttctaattc

SEQ ID NO: 323 - protein, 56 aa, Staphylococcus aureus
MLSFSQNRSHSLEQSLKEGYSQMADLNLSLANEAFPIECEACDCNETYLSSNSTNE

SEQ ID NO: 324 - DNA, 300 bp, Staphylococcus aureus
aatggcatggatgctcaaacatatggttctcaaggacagcaacgtacaacggctttgtccattaaattagctgaaattgagttaatgaatatcgaagttggggaatatcccatcttattattagacgatgtactcagtgaattagatgattcgcgtcaaacgcatttattaagtacgattcagcataaagtacaaacatttgtcactacgacatctgtagatggtattgatcatgaaatcatgaataacgctaaattgtatcgtattaatcaaggtgaaattataaagtaacagaaagcg

SEQ ID NO: 325 - DNA, 300 bp, Staphylococcus aureus
caaatgcagttaaacatgcatacaaagaaaataacaatgtgggcattattaacatatattttgaaattttagaagataaaattaaaattgttatttctgataaaggtgacagttttgattatgaaacaactaaatcaaaaataggtccttacgataaagacgaaaatatagactttttacgcgaaggtggcctaggtttatttttaatcgaatctttaatggatgaagtcacagtatataaagaatctggtgtgacaatcagtatgactaagtatataaaaaaagagcaggtgcgaaata

SEQ ID NO: 326 - DNA, 300 bp, Staphylococcus aureus
tatggtattgaagagttcttagaagtgaaatctatagctggatattttaaataaatttgatttttgaattaaaaatcgcaataaaacagtgcacatgactaattaagttttgtgtactgttttaattttgcaatttttataaatagattttgtaattaaaataaaaatttgctatagttattcatgtatttaaaaggttggggattagcataatgggattgtgctagcacagttatttatgcattgtcatgcctatctattacttactaactaaaaaataatgaaatgggtgtaaactat

SEQ ID NO: 327 - DNA, 243 bp, Artificial Sequence
  Promoter pTK3 forward
ttgcgaaatccattcctcttccactacaagcaccataattaaacaacaattcaatagaataagacttgcaaaacatagttatgtcgctatataaacgcctgcgaccaataaatcttttaaacataacataatgcaaaaacatcatttaacaatgctaaaaatgtctcttcaatacatgttgatagtaattaacttttaacgaacagttaattcgaaaacgcttacaaatggattattatatat

SEQ ID NO: 328 - DNA, 243 bp, Artificial Sequence
  Promoter pTK3 reverse
aacgctttaggtaaggagaaggtgatgttcgtggtattaatttgttgttaagttatcttattctgaacgttttgtatcaatacagcgatatatttgcggacgctggttatttagaaaatttgtattgtattacgtttttgtagtaaattgttacgatttttacagagaagttatgtacaactatcattaattgaaaattgcttgtcaattaagcttttgcgaatgtttacctaataatatata

SEQ ID NO: 329 - DNA, 31 bp, Artificial Sequence
  Primer TKO1
gatgcgcatgcttgcgaaatccattcctctt

SEQ ID NO: 330 - DNA, 52 bp, Artificial Sequence
  Primer DR_233
cgacggtatcgataagcttggccactggcgtcaaatactgtaatgaagaatg

SEQ ID NO: 331 - DNA, 46 bp, Artificial Sequence
  Primer DR_296
catctaattggacaaattctatgagagtagattttgttaatttaag

SEQ ID NO: 332 - DNA, 38 bp, Artificial Sequence
  Primer DR_280
gtagacgcaatacaaaataggtgacatatagccgcacc

SEQ ID NO: 333 - DNA, 53 bp, Artificial Sequence; identical to SEQ ID NO: 303
  Primer DR_236

SEQ ID NO: 334 - DNA, 57 bp, Artificial Sequence
  Primer DR_297
catagaatttgtccaattagatgtcccactacatcctgctaaaacaagtaggaaagc

SEQ ID NO: 335 - DNA, 32 bp, Artificial Sequence
  Primer DR_228
ctattttgtattgcgtctacttagccaataag

SEQ ID NO: 336 - DNA, 25 bp, Artificial Sequence
  Primer DR_022
caagcttatcgataccgtcgacctc

SEQ ID NO: 337 - DNA, 23 bp, Artificial Sequence
  Primer DR_023
gggatccactagttctagagcgg

SEQ ID NO: 338 - DNA, 29 bp, Artificial Sequence
  Primer DR_303
caagccaccaaagcacgtgcctatttgcc

SEQ ID NO: 339 - DNA, 48 bp, Artificial Sequence
  Primer DR_304
cagtgaaatagatagattggttgaaaaacaatcttcaaaagtcggacg